European Patent Specification EP 3 515 934 B1, published February 25, 2026. Title: COMPOSITIONS COMPRISING SASP MODULATORS AND SENESCENCE ATTENUATORS AND USES THEREOF FOR MODULATING  CELLULAR SENESCENCE. Applicant: RSEM, LIMITED PARTNERSHIP Sapieha, Przemyslaw Mallette, Frederick Antoine Oubaha, Malika Beaulieu, Normand Wilson, Ariel. The sequence listing filed with the application follows.

SEQUENCE LISTING (110 sequences)

SEQ ID NO: 1 - DNA, 22 bp, Artificial sequence
  Synthetic construct
gacggccaggtcatcactattg

SEQ ID NO: 2 - DNA, 21 bp, Artificial sequence
  Synthetic construct
ctggtacatcagcacctcaca

SEQ ID NO: 3 - DNA, 21 bp, Artificial sequence
  Synthetic construct
ctctgggaaatcgtggaaatg

SEQ ID NO: 4 - DNA, 22 bp, Artificial sequence
  Synthetic construct
ccgaacgtgatccgctacttct

SEQ ID NO: 5 - DNA, 20 bp, Artificial sequence
  Synthetic construct
ggccaatcccaagagcagag

SEQ ID NO: 6 - DNA, 20 bp, Artificial sequence
  Synthetic construct
ctccactgctgcttcctgag

SEQ ID NO: 7 - DNA, 21 bp, Artificial sequence
  Synthetic construct
ccgtgttggttcatccctgta

SEQ ID NO: 8 - DNA, 17 bp, Artificial sequence
  Synthetic construct
tgacgtcgtggaactgc

SEQ ID NO: 9 - DNA, 22 bp, Artificial sequence
  Synthetic construct
gggacttcgctatcttcagaac

SEQ ID NO: 10 - DNA, 20 bp, Artificial sequence
  Synthetic construct
ggactctccacctgcaagac

SEQ ID NO: 11 - DNA, 21 bp, Artificial sequence
  Synthetic construct
ctgagtccgaatcaggtccag

SEQ ID NO: 12 - DNA, 21 bp, Artificial sequence
  Synthetic construct
cgcgacgtggaactggcagaa

SEQ ID NO: 13 - DNA, 20 bp, Artificial sequence
  Synthetic construct
gccctgagtcaagaggacag

SEQ ID NO: 14 - DNA, 20 bp, Artificial sequence
  Synthetic construct
caaggcttttgaaggcaaag

SEQ ID NO: 15 - DNA, 20 bp, Artificial sequence
  Synthetic construct
gtcacagatgtgccgaatgg

SEQ ID NO: 16 - DNA, 20 bp, Artificial sequence
  Synthetic construct
ggcggtggtgacagtatctt

SEQ ID NO: 17 - DNA, 22 bp, Artificial sequence
  Synthetic construct
ccacaggattccatacccaaga

SEQ ID NO: 18 - DNA, 20 bp, Artificial sequence
  Synthetic construct
gagctccttaacatgccctg

SEQ ID NO: 19 - DNA, 24 bp, Artificial sequence
  Synthetic construct
aagtgcatcatcgttgttcataca

SEQ ID NO: 20 - DNA, 22 bp, Artificial sequence
  Synthetic construct
cgcaaagtccttctgctccaca

SEQ ID NO: 21 - DNA, 20 bp, Artificial sequence
  Synthetic construct
gccacatgctagacacgcta

SEQ ID NO: 22 - DNA, 20 bp, Artificial sequence
  Synthetic construct
tgctgagctcatgccctttg

SEQ ID NO: 23 - DNA, 29 bp, Artificial sequence
  Synthetic construct
ttttggatttttaagacagagtctttgta

SEQ ID NO: 24 - DNA, 20 bp, Artificial sequence
  Synthetic construct
gaaagacttgtgaagtcggc

SEQ ID NO: 25 - DNA, 21 bp, Artificial sequence
  Synthetic construct
ggcgtgcttttaggaatgttg

SEQ ID NO: 26 - DNA, 20 bp, Artificial sequence
  Synthetic construct
catagatggcgttgttgcgg

SEQ ID NO: 27 - DNA, 21 bp, Artificial sequence
  Synthetic construct
gtccatgggaagatgttctgg

SEQ ID NO: 28 - DNA, 24 bp, Artificial sequence
  Synthetic construct
cttggtggtttgctacgacgtggg

SEQ ID NO: 29 - DNA, 20 bp, Artificial sequence
  Synthetic construct
ctcctaggcccctcagaagt

SEQ ID NO: 30 - DNA, 20 bp, Artificial sequence
  Synthetic construct
agaaggtgtttgtggctgct

SEQ ID NO: 31 - DNA, 20 bp, Artificial sequence
  Synthetic construct
tgagcgtgatcagctccagg

SEQ ID NO: 32 - DNA, 20 bp, Artificial sequence
  Synthetic construct
gtcactgacagaggcgatga

SEQ ID NO: 33 - DNA, 21 bp, Artificial sequence
  Synthetic construct
aaatccttgatattaaccagg

SEQ ID NO: 34 - DNA, 21 bp, Artificial sequence
  Synthetic construct
tttcccgtaaatatcacaccg

SEQ ID NO: 35 - DNA, 21 bp, Artificial sequence
  Synthetic construct
ttgaaactactttaagaacgg

SEQ ID NO: 36 - DNA, 21 bp, Artificial sequence
  Synthetic construct
aaattagcacattctttcagg

SEQ ID NO: 37 - DNA, 21 bp, Artificial sequence
  Synthetic construct
aaattgccaatataccaaggc

SEQ ID NO: 38 - DNA, 21 bp, Artificial sequence
  Synthetic construct
aatgagctgcatgaagtctcg

SEQ ID NO: 39 - DNA, 21 bp, Artificial sequence
  Synthetic construct
aaattggcacattctttcagg

SEQ ID NO: 40 - DNA, 21 bp, Artificial sequence
  Synthetic construct
ttcattaggaatacatcctgc

SEQ ID NO: 41 - DNA, 21 bp, Artificial sequence
  Synthetic construct
ttatttataggaaacactggg

SEQ ID NO: 42 - DNA, 19 bp, Artificial sequence
  Synthetic construct
aacgccacccatccaacca

SEQ ID NO: 43 - DNA, 22 bp, Artificial sequence
  Synthetic construct
gcaagctgaccctgaagttcat

SEQ ID NO: 44 - protein, 644 aa, Homo sapiens
MERGLPLLCAVLALVLAPAGAFRNDKCGDTIKIESPGYLTSPGYPHSYHPSEKCEWLIQAPDPYQRIMINFNPHFDLEDRDCKYDYVEVFDGENENGHFRGKFCGKIAPPPVVSSGPFLFIKFVSDYETHGAGFSIRYEIFKRGPECSQNYTTPSGVIKSPGFPEKYPNSLECTYIVFVPKMSEIILEFESFDLEPDSNPPGGMFCRYDRLEIWDGFPDVGPHIGRYCGQKTPGRIRSSSGILSMVFYTDSAIAKEGFSANYSVLQSSVSEDFKCMEALGMESGEIHSDQITASSQYSTNWSAERSRLNYPENGWTPGEDSYREWIQVDLGLLRFVTAVGTQGAISKETKKKYYVKTYKIDVSSNGEDWITIKEGNKPVLFQGNTNPTDVVVAVFPKPLITRFVRIKPATWETGISMRFEVYGCKITDYPCSGMLGMVSGLISDSQITSSNQGDRNWMPENIRLVTSRSGWALPPAPHSYINEWLQIDLGEEKIVRGIIIQGGKHRENKVFMRKFKIGYSNNGSDWKMIMDDSKRKAKSFEGNNNYDTPELRTFPALSTRFIRIYPERATHGGLGLRMELLGCEVEAPTAGPTTPNGNLVDECDDDQANCHSGTGDDFQLTGGTTVLATEKPTVIDSTIQSGIK

SEQ ID NO: 45 - protein, 609 aa, Homo sapiens
MERGLPLLCAVLALVLAPAGAFRNDKCGDTIKIESPGYLTSPGYPHSYHPSEKCEWLIQAPDPYQRIMINFNPHFDLEDRDCKYDYVEVFDGENENGHFRGKFCGKIAPPPVVSSGPFLFIKFVSDYETHGAGFSIRYEIFKRGPECSQNYTTPSGVIKSPGFPEKYPNSLECTYIVFVPKMSEIILEFESFDLEPDSNPPGGMFCRYDRLEIWDGFPDVGPHIGRYCGQKTPGRIRSSSGILSMVFYTDSAIAKEGFSANYSVLQSSVSEDFKCMEALGMESGEIHSDQITASSQYSTNWSAERSRLNYPENGWTPGEDSYREWIQVDLGLLRFVTAVGTQGAISKETKKKYYVKTYKIDVSSNGEDWITIKEGNKPVLFQGNTNPTDVVVAVFPKPLITRFVRIKPATWETGISMRFEVYGCKITDYPCSGMLGMVSGLISDSQITSSNQGDRNWMPENIRLVTSRSGWALPPAPHSYINEWLQIDLGEEKIVRGIIIQGGKHRENKVFMRKFKIGYSNNGSDWKMIMDDSKRKAKSFEGNNNYDTPELRTFPALSTRFIRIYPERATHGGLGLRMELLGCEVEGGTTVLATEKPTVIDSTIQSGIK

SEQ ID NO: 46 - protein, 704 aa, Homo sapiens
MERGLPLLCAVLALVLAPAGAFRNDKCGDTIKIESPGYLTSPGYPHSYHPSEKCEWLIQAPDPYQRIMINFNPHFDLEDRDCKYDYVEVFDGENENGHFRGKFCGKIAPPPVVSSGPFLFIKFVSDYETHGAGFSIRYEIFKRGPECSQNYTTPSGVIKSPGFPEKYPNSLECTYIVFVPKMSEIILEFESFDLEPDSNPPGGMFCRYDRLEIWDGFPDVGPHIGRYCGQKTPGRIRSSSGILSMVFYTDSAIAKEGFSANYSVLQSSVSEDFKCMEALGMESGEIHSDQITASSQYSTNWSAERSRLNYPENGWTPGEDSYREWIQVDLGLLRFVTAVGTQGAISKETKKKYYVKTYKIDVSSNGEDWITIKEGNKPVLFQGNTNPTDVVVAVFPKPLITRFVRIKPATWETGISMRFEVYGCKITDYPCSGMLGMVSGLISDSQITSSNQGDRNWMPENIRLVTSRSGWALPPAPHSYINEWLQIDLGEEKIVRGIIIQGGKHRENKVFMRKFKIGYSNNGSDWKMIMDDSKRKAKSFEGNNNYDTPELRTFPALSTRFIRIYPERATHGGLGLRMELLGCEVEAPTAGPTTPNGNLVDECDDDQANCHSGTGDDFQLTGAETIFIPLLYHFSSCLSWDQLTPVCVLVTPHGRELPRNRSCLARTRASSFPHVIWIDELFLIATTICNNNLSHFESQRLGLS

SEQ ID NO: 47 - protein, 923 aa, artificial sequence
  Synthetic construct
  VARIANT (11)..(11): X is any amino acid
  VARIANT (15)..(15): X is any amino acid
  VARIANT (18)..(18): X is any amino acid
  VARIANT (24)..(24): X is any amino acid
  VARIANT (29)..(29): X is any amino acid
  VARIANT (35)..(35): X is any amino acid
  VARIANT (62)..(62): X is any amino acid
  VARIANT (90)..(90): X is any amino acid
  VARIANT (96)..(96): X is any amino acid
  VARIANT (98)..(98): X is any amino acid
  VARIANT (99)..(99): X is any amino acid
  VARIANT (100)..(100): X is any amino acid
  VARIANT (100)..(100): X is any amino acid
  VARIANT (110)..(110): X is any amino acid
  VARIANT (140)..(140): X is any amino acid
  VARIANT (153)..(153): X is any amino acid
  VARIANT (155)..(155): X is any amino acid
  VARIANT (170)..(170): X is any amino acid
  VARIANT (170)..(170): X is any amino acid
  VARIANT (177)..(177): X is any amino acid
  VARIANT (196)..(196): X is any amino acid
  VARIANT (204)..(204): X is any amino acid
  VARIANT (219)..(219): X is any amino acid
  VARIANT (242)..(242): X is any amino acid
  VARIANT (269)..(269): X is any amino acid
  VARIANT (298)..(298): X is any amino acid
  VARIANT (303)..(303): X is any amino acid
  VARIANT (323)..(323): X is any amino acid
  VARIANT (359)..(359): X is any amino acid
  VARIANT (360)..(360): X is any amino acid
  VARIANT (362)..(362): X is any amino acid
  VARIANT (371)..(371): X is any amino acid
  VARIANT (372)..(372): X is any amino acid
  VARIANT (378)..(378): X is any amino acid
  VARIANT (379)..(379): X is any amino acid
  VARIANT (380)..(380): X is any amino acid
  VARIANT (392)..(392): X is any amino acid
  VARIANT (393)..(393): X is any amino acid
  VARIANT (393)..(393): X is any amino acid
  VARIANT (396)..(396): X is any amino acid
  VARIANT (409)..(409): X is any amino acid
  VARIANT (410)..(410): X is any amino acid
  VARIANT (449)..(449): X is any amino acid
  VARIANT (453)..(453): X is any amino acid
  VARIANT (469)..(469): X is any amino acid
  VARIANT (476)..(476): X is any amino acid
  VARIANT (479)..(479): X is any amino acid
  VARIANT (481)..(481): X is any amino acid
  VARIANT (487)..(487): X is any amino acid
  VARIANT (491)..(491): X is any amino acid
  VARIANT (498)..(498): X is any amino acid
  VARIANT (518)..(518): X is any amino acid
  VARIANT (518)..(518): X is any amino acid
  VARIANT (518)..(518): X is any amino acid
  VARIANT (528)..(528): X is any amino acid
  VARIANT (528)..(528): X is any amino acid
  VARIANT (553)..(553): X is any amino acid
  VARIANT (553)..(553): X is any amino acid
  VARIANT (555)..(555): X is any amino acid
  VARIANT (556)..(556): X is any amino acid
  VARIANT (572)..(572): X is any amino acid
  VARIANT (587)..(587): X is any amino acid
  VARIANT (599)..(599): X is any amino acid
  VARIANT (601)..(601): X is any amino acid
  VARIANT (634)..(634): X is any amino acid
  VARIANT (634)..(634): X is any amino acid
  VARIANT (667)..(667): X is any amino acid
  VARIANT (669)..(669): X is any amino acid
  VARIANT (672)..(672): X is any amino acid
  VARIANT (674)..(674): X is any amino acid
  VARIANT (717)..(717): X is any amino acid
  VARIANT (741)..(741): X is any amino acid
  VARIANT (755)..(755): X is any amino acid
  VARIANT (756)..(756): X is any amino acid
  VARIANT (805)..(805): X is any amino acid
  VARIANT (813)..(813): X is any amino acid
  VARIANT (820)..(820): X is any amino acid
  VARIANT (835)..(835): X is any amino acid
  VARIANT (838)..(838): X is any amino acid
  VARIANT (916)..(916): X is any amino acid
  VARIANT (919)..(919): X is any amino acid
MERGLPLLCAXLALXLAXAGAFRXDKCGXTIKIEXPGYLTSPGYPHSYHPSEKCEWLIQAPXPYQRIMINFNPHFDLEDRDCKYDYVEVXDGENEXGXXXGKFCGKIAPXPVVSSGPFLFIKFVSDYETHGAGFSIRYEXFKRGPECSQNYTXPXGVIKSPGFPEKYPNSLECTYIXFAPKMSEIILEFESFDLEXDSNPPGGXFCRYDRLEIWDGFPXVGPHIGRYCGQKTPGRIRSSSGXLSMVFYTDSAIAKEGFSANYSVLQSSXSEDFKCMEALGMESGEIHSDQITASSQYXTNWSXERSRLNYPENGWTPGEDSYXEWIQVDLGLLRFVTAVGTQGAISKETKKKYYVKTYXXDXSSNGEDWIXXKEGNKXXXFQGNTNPTDVVXXVFXKPLITRFVRIKPXXWETGISMRFEVYGCKITDYPCSGMLGMVSGLISDSQITXSNQXDRNWMPENIRLVTSRXGWALPPXPHXYXNEWLQXDLGXEKIVRGXIIQGGKHRENKVFMRKFKIXYSNNGSDWKXIMDDSKRKAKSFEGNNNYDTPELRXFXXLSTRFIRIYPERATHXGLGLRMELLGCEVEXPTAGPTTPNGNXVDECDDDQANCHSGTGDDFQLTGGTTVLATEKPTXIDSTIQSEFPTYGFNCEFGWGSHKTFCHWEHDXHXQLXWXVLTSKTGPIQDHTGDGNFIYSQADENQKGKVARLVSPVVYSQXSAHCMTFWYHMSGSHVGTLRVKLXYQKPEEYDQLVWMXXGHQGDHWKEGRVLLHKSLKLYQVIFEGEIGKGNLGGIAVDDISINNHIXQEDCAKPXLDKKNNXEIKIDETGSTPGYEXEGXGDKNISRKPGNVLKTLDPILITIIAMSALGVLLGAVCGVVLYCACWHNGMSERNLSALENYNFELVDGVKLKKDKLNXQSXYSEA

SEQ ID NO: 48 - protein, 923 aa, Mus musculus
MERGLPLLCATLALALALAGAFRSDKCGGTIKIENPGYLTSPGYPHSYHPSEKCEWLIQAPEPYQRIMINFNPHFDLEDRDCKYDYVEVIDGENEGGRLWGKFCGKIAPSPVVSSGPFLFIKFVSDYETHGAGFSIRYEIFKRGPECSQNYTAPTGVIKSPGFPEKYPNSLECTYIIFAPKMSEIILEFESFDLEQDSNPPGGMFCRYDRLEIWDGFPEVGPHIGRYCGQKTPGRIRSSSGVLSMVFYTDSAIAKEGFSANYSVLQSSISEDFKCMEALGMESGEIHSDQITASSQYGTNWSVERSRLNYPENGWTPGEDSYKEWIQVDLGLLRFVTAVGTQGAISKETKKKYYVKTYRVDISSNGEDWISLKEGNKAIIFQGNTNPTDVVLGVFSKPLITRFVRIKPVSWETGISMRFEVYGCKITDYPCSGMLGMVSGLISDSQITASNQADRNWMPENIRLVTSRTGWALPPSPHPYTNEWLQVDLGDEKIVRGVIIQGGKHRENKVFMRKFKIAYSNNGSDWKTIMDDSKRKAKSFEGNNNYDTPELRTFSPLSTRFIRIYPERATHSGLGLRMELLGCEVEAPTAGPTTPNGNPVDECDDDQANCHSGTGDDFQLTGGTTVLATEKPTIIDSTIQSEFPTYGFNCEFGWGSHKTFCHWEHDSHAQLRWSVLTSKTGPIQDHTGDGNFIYSQADENQKGKVARLVSPVVYSQSSAHCMTFWYHMSGSHVGTLRVKLRYQKPEEYDQLVWMVVGHQGDHWKEGRVLLHKSLKLYQVIFEGEIGKGNLGGIAVDDISINNHISQEDCAKPTDLDKKNTEIKIDETGSTPGYEGEGEGDKNISRKPGNVLKTLDPILITIIAMSALGVLLGAVCGVVLYCACWHNGMSERNLSALENYNFELVDGVKLKKDKLNPQSNYSEA

SEQ ID NO: 49 - protein, 922 aa, Ratus norvegicus
MERGLPLLCATLALALALAGAFRSDKCGGTIKIENPGYLTSPGYPHSYHPSEKCEWLIQAPEPYQRIMINFNPHFDLEDRDCKYDYVEVIDGENEGGRLWGKFCGKIAPSPVVSSGPFLFIKFVSDYETHGAGFSIRYEIFKRGPECSQNYTAPTGVIKSPGFPEKYPNSLECTYIIFAPKMSEIILEFESFDLEQDSNPPGGVFCRYDRLEIWDGFPEVGPHIGRYCGQKTPGRIRSSSGILSMVFYTDSAIAKEGFSANYSVLQSSISEDFKCMEALGMESGEIHSDQITASSQYGTNWSVERSRLNYPENGWTPGEDSYREWIQVDLGLLRFVTAVGTQGAISKETKKKYYVKTYRVDISSNGEDWITLKEGNKAIIFQGNTNPTDVVFGVFPKPLITRFVRIKPASWETGISMRFEVYGCKITDYPCSGMLGMVSGLISDSQITASNQGDRNWMPENIRLVTSRTGWALPPSPHPYINEWLQVDLGDEKIVRGVIIQGGKHRENKVFMRKFKIAYSNNGSDWKMIMDDSKRKAKSFEGNNNYDTPELRAFTPLSTRFIRIYPERATHSGLGLRMELLGCEVEVPTAGPTTPNGNPVDECDDDQANCHSGTGDDFQLTGGTTVLATEKPTIIDSTIQSEFPTYGFNCEFGWGSHKTFCHWEHDSHAQLRWRVLTSKTGPIQDHTGDGNFIYSQADENQKGKVARLVSPVVYSQSSAHCMTFWYHMSGSHVGTLRVKLHYQKPEEYDQLVWMVVGHQGDHWKEGRVLLHKSLKLYQVIFEGEIGKGNLGGIAVDDISINNHIPQEDCAKPTDLDKKNTEIKIDETGSTPGYEEGKGDKNISRKPGNVLKTLDPILITIIAMSALGVLLGAVCGVVLYCACWHNGMSERNLSALENYNFELVDGVKLKKDKLNPQSNYSEA

SEQ ID NO: 50 - protein, 771 aa, Homo sapiens [sequence omitted]

SEQ ID NO: 51 - DNA, 1308 bp, artificial sequence
  Synthetic construct
atggagagggggctgccgctcctctgcgccgtgctcgccctcgtcctcgccccggccggcgcttttcgcaacgataaatgtggcgatactataaaaattgaaagccccgggtaccttacatctcctggttatcctcattcttatcacccaagtgaaaaatgcgaatggctgattcaggctccggacccataccagagaattatgatcaacttcaaccctcacttcgatttggaggacagagactgcaagtatgactacgtggaagtcttcgatggagaaaatgaaaatggacattttaggggaaagttctgtggaaagatagcccctcctcctgttgtgtcttcagggccatttctttttatcaaatttgtctctgactacgaaacacatggtgcaggattttccatacgttatgaacttttcaagagaggtcctgaatgttcccagaactacacaacacctagtggagtgataaagtcccccggattccctgaaaaatatcccaacagccttgaatgcacttatattgtctttgcgccaaagatgtcagagattatcctggaatttgaaagctttgacctggagcctgactcaaatcctccaggggggatgttctgtcgctacgaccggctagaaatctgggatggattccctgatgttggccctcacattgggcgttactgtggacagaaaacaccaggtcgaatccgatcctcatcgggcattctctccatggttttttacaccgacagcgcgatagcaaaagaaggtttctcagcaaactacagtgtcttgcagagcagtgtctcagaagatttcaaatgtatggaagctctgggcatggaatcaggagaaattcattctgaccagatcacagcttcttcccagtatagcaccaactggtctgcagagcgctcccgcctgaactaccctgagaatgggtggactcccggagagaagtcctaccgagagtggatacaggtagacttgggccttctgcgctttgtcacggctgtcgggacacagggcgccatttcaaaagaaaccaagaagaaatattatgtcaagacttacaagatcgacgttagctccaacggggaagactggatcaccataaaagaaggaaacaaacctgttctctttcagggaaacaccaaccctacagatgttgtggttgcagtattccccaaaccactgataactcgatttgtccgaatcaagcctgcaacttgggaaactggcatatctatgagatttgaagtatatggttgcagatctggatccaaggaaaacttgtatttccagggc

SEQ ID NO: 52 - protein, 436 aa, artificial sequence
  Synthetic construct
MERGLPLLCAVLALVLAPAGAFRNDKCGDTIKIESPGYLTSPGYPHSYHPSEKCEWLIQAPDPYQRIMINFNPHFDLEDRDCKYDYVEVFDGENENGHFRGKFCGKIAPPPVVSSGPFLFIKFVSDYETHGAGFSIRYELFKRGPECSQNYTTPSGVIKSPGFPEKYPNSLECTYIVFAPKMSEIILEFESFDLEPDSNPPGGMFCRYDRLEIWDGFPDVGPHIGRYCGQKTPGRIRSSSGILSMVFYTDSAIAKEGFSANYSVLQSSVSEDFKCMEALGMESGEIHSDQITASSQYSTNWSAERSRLNYPENGWTPGEKSYREWIQVDLGLLRFVTAVGTQGAISKETKKKYYVKTYKIDVSSNGEDWITIKEGNKPVLFQGNTNPTDVVVAVFPKPLITRFVRIKPATWETGISMRFEVYGCRSGSKENLYFQG

SEQ ID NO: 53 - DNA, 1785 bp, artificial sequence
  Synthetic construct
atggagagggggctgccgctcctctgcgccgtgctcgccctcgtcctcgccccggccggcgcttttcgcaacgataaatgtggcgatactataaaaattgaaagccccgggtaccttacatctcctggttatcctcattcttatcacccaagtgaaaaatgcgaatggctgattcaggctccggacccataccagagaattatgatcaacttcaaccctcacttcgatttggaggacagagactgcaagtatgactacgtggaagtcttcgatggagaaaatgaaaatggacattttaggggaaagttctgtggaaagatagcccctcctcctgttgtgtcttcagggccatttctttttatcaaatttgtctctgactacgaaacacatggtgcaggattttccatacgttatgaacttttcaagagaggtcctgaatgttcccagaactacacaacacctagtggagtgataaagtcccccggattccctgaaaaatatcccaacagccttgaatgcacttatattgtctttgcgccaaagatgtcagagattatcctggaatttgaaagctttgacctggagcctgactcaaatcctccaggggggatgttctgtcgctacgaccggctagaaatctgggatggattccctgatgttggccctcacattgggcgttactgtggacagaaaacaccaggtcgaatccgatcctcatcgggcattctctccatggttttttacaccgacagcgcgatagcaaaagaaggtttctcagcaaactacagtgtcttgcagagcagtgtctcagaagatttcaaatgtatggaagctctgggcatggaatcaggagaaattcattctgaccagatcacagcttcttcccagtatagcaccaactggtctgcagagcgctcccgcctgaactaccctgagaatgggtggactcccggagagaagtcctaccgagagtggatacaggtagacttgggccttctgcgctttgtcacggctgtcgggacacagggcgccatttcaaaagaaaccaagaagaaatattatgtcaagacttacaagatcgacgttagctccaacggggaagactggatcaccataaaagaaggaaacaaacctgttctctttcagggaaacaccaaccctacagatgttgtggttgcagtattccccaaaccactgataactcgatttgtccgaatcaagcctgcaacttgggaaactggcatatctatgagatttgaagtatatggttgcaagataacagattatccttgctctggaatgttgggtatggtgtctggacttatttctgactcccagatcacatcatccaaccaaggggacagaaactggatgcctgaaaacatccgcctggtaaccagtcgctctggctgggcacttccacccgcacctcattcctacatcaatgagtggctccaaatagacctgggggaggagaagatcgtgaggggcatcatcattcagggtgggaagcaccgagagaacaaggtgttcatgaggaagttcaagatcgggtacagcaacaacggctcggactggaagatgatcatggatgacagcaaacgcaaggcgaagtcttttgagggcaacaacaactatgatacacctgagctgcggacttttccagctctctccacgcgattcatcaggatctaccccgagagagccactcatggcggactggggctcagaatggagctgctgggctgtagatctggatccaaggaaaacttgtatttccagggc

SEQ ID NO: 54 - protein, 595 aa, artificial sequence
  Synthetic construct
MERGLPLLCAVLALVLAPAGAFRNDKCGDTIKIESPGYLTSPGYPHSYHPSEKCEWLIQAPDPYQRIMINFNPHFDLEDRDCKYDYVEVFDGENENGHFRGKFCGKIAPPPVVSSGPFLFIKFVSDYETHGAGFSIRYELFKRGPECSQNYTTPSGVIKSPGFPEKYPNSLECTYIVFAPKMSEIILEFESFDLEPDSNPPGGMFCRYDRLEIWDGFPDVGPHIGRYCGQKTPGRIRSSSGILSMVFYTDSAIAKEGFSANYSVLQSSVSEDFKCMEALGMESGEIHSDQITASSQYSTNWSAERSRLNYPENGWTPGEKSYREWIQVDLGLLRFVTAVGTQGAISKETKKKYYVKTYKIDVSSNGEDWITIKEGNKPVLFQGNTNPTDVVVAVFPKPLITRFVRIKPATWETGISMRFEVYGCKITDYPCSGMLGMVSGLISDSQITSSNQGDRNWMPENIRLVTSRSGWALPPAPHSYINEWLQIDLGEEKIVRGIIIQGGKHRENKVFMRKFKIGYSNNGSDWKMIMDDSKRKAKSFEGNNNYDTPELRTFPALSTRFIRIYPERATHGGLGLRMELLGCRSGSKENLYFQG

SEQ ID NO: 55 - DNA, 2154 bp, artificial sequence
  Synthetic construct
atggagagggggctgccgctcctctgcgccgtgctcgccctcgtcctcgccccggccggcgcttttcgcaacgataaatgtggcgatactataaaaattgaaagccccgggtaccttacatctcctggttatcctcattcttatcacccaagtgaaaaatgcgaatggctgattcaggctccggacccataccagagaattatgatcaacttcaaccctcacttcgatttggaggacagagactgcaagtatgactacgtggaagtcttcgatggagaaaatgaaaatggacattttaggggaaagttctgtggaaagatagcccctcctcctgttgtgtcttcagggccatttctttttatcaaatttgtctctgactacgaaacacatggtgcaggattttccatacgttatgaacttttcaagagaggtcctgaatgttcccagaactacacaacacctagtggagtgataaagtcccccggattccctgaaaaatatcccaacagccttgaatgcacttatattgtctttgcgccaaagatgtcagagattatcctggaatttgaaagctttgacctggagcctgactcaaatcctccaggggggatgttctgtcgctacgaccggctagaaatctgggatggattccctgatgttggccctcacattgggcgttactgtggacagaaaacaccaggtcgaatccgatcctcatcgggcattctctccatggttttttacaccgacagcgcgatagcaaaagaaggtttctcagcaaactacagtgtcttgcagagcagtgtctcagaagatttcaaaaagataacagattatccttgctctggaatgttgggtatggtgtctggacttatttctgactcccagatcacatcatccaaccaaggggacagaaactggatgcctgaaaacatccgcctggtaaccagtcgctctggctgggcacttccacccgcacctcattcctacatcaatgagtggctccaaatagacctgggggaggagaagatcgtgaggggcatcatcattcagggtgggaagcaccgagagaacaaggtgttcatgaggaagttcaagatcgggtacagcaacaacggctcggactggaagatgatcatggatgacagcaaacgcaaggcgaagtcttttgagggcaacaacaactatgatacacctgagctgcggacttttccagctctctccacgcgattcatcaggatctaccccgagagagccactcatggcggactggggctcagaatggagctgctgggctgtgaagtggaagcccctacagctggaccgaccactcccaacgggaacttggtggatgaatgtgatgacgaccaggccaactgccacagtggaacaggtgatgacttccagctcacaggtggcaccactgtgctggccacagaaaagcccacggtcatagacagcaccatacaatcagagtttccaacatatggttttaactgtgaatttggctggggctctcacaagaccttctgccactgggaacatgacaatcacgtgcagctcaagtggagtgtgttgaccagcaagacgggacccattcaggatcacacaggagatggcaacttcatctattcccaagctgacgaaaatcagaagggcaaagtggctcgcctggtgagccctgtggtttattcccagaactctgcccactgcatgaccttctggtatcacatgtctgggtcccacgtcggcacactcagggtcaaactgcgctaccagaagccagaggagtacgatcagctggtctggatggccattggacaccaaggtgaccactggaaggaagggcgtgtcttgctccacaagtctctgaaactttatcaggtgattttcgagggcgaaatcggaaaaggaaaccttggtgggattgctgtggatgacattagtattaataaccacatttcacaagaagattgtgcaaaaccagcagacctggataaaaagaacccagaaattaaaattgatgaaacagggagcacgccaggatacgaaggtgaaggagaaggtgacaagaacatctccaggaagccaggcaatgtgttgaagaccttagaccccagatctggatccaaggaaaacttgtatttccagggc

SEQ ID NO: 56 - protein, 718 aa, artificial sequence
  Synthetic construct
MERGLPLLCAVLALVLAPAGAFRNDKCGDTIKIESPGYLTSPGYPHSYHPSEKCEWLIQAPDPYQRIMINFNPHFDLEDRDCKYDYVEVFDGENENGHFRGKFCGKIAPPPVVSSGPFLFIKFVSDYETHGAGFSIRYELFKRGPECSQNYTTPSGVIKSPGFPEKYPNSLECTYIVFAPKMSEIILEFESFDLEPDSNPPGGMFCRYDRLEIWDGFPDVGPHIGRYCGQKTPGRIRSSSGILSMVFYTDSAIAKEGFSANYSVLQSSVSEDFKKITDYPCSGMLGMVSGLISDSQITSSNQGDRNWMPENIRLVTSRSGWALPPAPHSYINEWLQIDLGEEKIVRGIIIQGGKHRENKVFMRKFKIGYSNNGSDWKMIMDDSKRKAKSFEGNNNYDTPELRTFPALSTRFIRIYPERATHGGLGLRMELLGCEVEAPTAGPTTPNGNLVDECDDDQANCHSGTGDDFQLTGGTTVLATEKPTVIDSTIQSEFPTYGFNCEFGWGSHKTFCHWEHDNHVQLKWSVLTSKTGPIQDHTGDGNFIYSQADENQKGKVARLVSPVVYSQNSAHCMTFWYHMSGSHVGTLRVKLRYQKPEEYDQLVWMAIGHQGDHWKEGRVLLHKSLKLYQVIFEGEIGKGNLGGIAVDDISINNHISQEDCAKPADLDKKNPEIKIDETGSTPGYEGEGEGDKNISRKPGNVLKTLDPRSGSKENLYFQG

SEQ ID NO: 57 - DNA, 1335 bp, artificial sequence
  Synthetic construct
atggagagggggctgccgctcctctgcgccgtgctcgccctcgtcctcgccccggccggcgcttttcgcaacgataaatgtggcgatactataaaaattgaaagccccgggtaccttacatctcctggttatcctcattcttatcacccaagtgaaaaatgcgaatggctgattcaggctccggacccataccagagaattatgatcaacttcaaccctcacttcgatttggaggacagagactgcaagtatgactacgtggaagtcttcgatggagaaaatgaaaatggacattttaggggaaagttctgtggaaagatagcccctcctcctgttgtgtcttcagggccatttctttttatcaaatttgtctctgactacgaaacacatggtgcaggattttccatacgttatgaacttttcaagagaggtcctgaatgttcccagaactacacaacacctagtggagtgataaagtcccccggattccctgaaaaatatcccaacagccttgaatgcacttatattgtctttgcgccaaagatgtcagagattatcctggaatttgaaagctttgacctggagcctgactcaaatcctccaggggggatgttctgtcgctacgaccggctagaaatctgggatggattccctgatgttggccctcacattgggcgttactgtggacagaaaacaccaggtcgaatccgatcctcatcgggcattctctccatggttttttacaccgacagcgcgatagcaaaagaaggtttctcagcaaactacagtgtcttgcagagcagtgtctcagaagatttcaaaaagataacagattatccttgctctggaatgttgggtatggtgtctggacttatttctgactcccagatcacatcatccaaccaaggggacagaaactggatgcctgaaaacatccgcctggtaaccagtcgctctggctgggcacttccacccgcacctcattcctacatcaatgagtggctccaaatagacctgggggaggagaagatcgtgaggggcatcatcattcagggtgggaagcaccgagagaacaaggtgttcatgaggaagttcaagatcgggtacagcaacaacggctcggactggaagatgatcatggatgacagcaaacgcaaggcgaagtcttttgagggcaacaacaactatgatacacctgagctgcggacttttccagctctctccacgcgattcatcaggatctaccccgagagagccactcatggcggactggggctcagaatggagctgctgggctgtagatctggatccaaggaaaacttgtatttccagggc

SEQ ID NO: 58 - protein, 445 aa, artificial sequence
  Synthetic construct
MERGLPLLCAVLALVLAPAGAFRNDKCGDTIKIESPGYLTSPGYPHSYHPSEKCEWLIQAPDPYQRIMINFNPHFDLEDRDCKYDYVEVFDGENENGHFRGKFCGKIAPPPVVSSGPFLFIKFVSDYETHGAGFSIRYELFKRGPECSQNYTTPSGVIKSPGFPEKYPNSLECTYIVFAPKMSEIILEFESFDLEPDSNPPGGMFCRYDRLEIWDGFPDVGPHIGRYCGQKTPGRIRSSSGILSMVFYTDSAIAKEGFSANYSVLQSSVSEDFKKITDYPCSGMLGMVSGLISDSQITSSNQGDRNWMPENIRLVTSRSGWALPPAPHSYINEWLQIDLGEEKIVRGIIIQGGKHRENKVFMRKFKIGYSNNGSDWKMIMDDSKRKAKSFEGNNNYDTPELRTFPALSTRFIRIYPERATHGGLGLRMELLGCRSGSKENLYFQG

SEQ ID NO: 59 - DNA, 2256 bp, artificial sequence
  Synthetic construct
atggagagggggctgccgctcctctgcgccgtgctcgccctcgtcctcgccccggccggcgcttttcgcaacgataaaagaggtcctgaatgttcccagaactacacaacacctagtggagtgataaagtcccccggattccctgaaaaatatcccaacagccttgaatgcacttatattgtctttgcgccaaagatgtcagagattatcctggaatttgaaagctttgacctggagcctgactcaaatcctccaggggggatgttctgtcgctacgaccggctagaaatctgggatggattccctgatgttggccctcacattgggcgttactgtggacagaaaacaccaggtcgaatccgatcctcatcgggcattctctccatggttttttacaccgacagcgcgatagcaaaagaaggtttctcagcaaactacagtgtcttgcagagcagtgtctcagaagatttcaaatgtatggaagctctgggcatggaatcaggagaaattcattctgaccagatcacagcttcttcccagtatagcaccaactggtctgcagagcgctcccgcctgaactaccctgagaatgggtggactcccggagaggattcctaccgagagtggatacaggtagacttgggccttctgcgctttgtcacggctgtcgggacacagggcgccatttcaaaagaaaccaagaagaaatattatgtcaagacttacaagatcgacgttagctccaacggggaagactggatcaccataaaagaaggaaacaaacctgttctctttcagggaaacaccaaccctacagatgttgtggttgcagtattccccaaaccactgataactcgatttgtccgaatcaagcctgcaacttgggaaactggcatatctatgagatttgaagtatatggttgcaagataacagattatccttgctctggaatgttgggtatggtgtctggacttatttctgactcccagatcacatcatccaaccaaggggacagaaactggatgcctgaaaacatccgcctggtaaccagtcgctctggctgggcacttccacccgcacctcattcctacatcaatgagtggctccaaatagacctgggggaggagaagatcgtgaggggcatcatcattcagggtgggaagcaccgagagaacaaggtgttcatgaggaagttcaagatcgggtacagcaacaacggctcggactggaagatgatcatggatgacagcaaacgcaaggcgaagtcttttgagggcaacaacaactatgatacacctgagctgcggacttttccagctctctccacgcgattcatcaggatctaccccgagagagccactcatggcggactggggctcagaatggagctgctgggctgtgaagtggaagcccctacagctggaccgaccactcccaacgggaacttggtggatgaatgtgatgacgaccaggccaactgccacagtggaacaggtgatgacttccagctcacaggtggcaccactgtgctggccacagaaaagcccacggtcatagacagcaccatacaatcagagtttccaacatatggttttaactgtgaatttggctggggctctcacaagaccttctgccactgggaacatgacaatcacgtgcagctcaagtggagtgtgttgaccagcaagacgggacccattcaggatcacacaggagatggcaacttcatctattcccaagctgacgaaaatcagaagggcaaagtggctcgcctggtgagccctgtggtttattcccagaactctgcccactgcatgaccttctggtatcacatgtctgggtcccacgtcggcacactcagggtcaaactgcgctaccagaagccagaggagtacgatcagctggtctggatggccattggacaccaaggtgaccactggaaggaagggcgtgtcttgctccacaagtctctgaaactttatcaggtgattttcgagggcgaaatcggaaaaggaaaccttggtgggattgctgtggatgacattagtattaataaccacatttcacaagaagattgtgcaaaaccagcagacctggataaaaagaacccagaaattaaaattgatgaaacagggagcacgccaggatacgaaggtgaaggagaaggtgacaagaacatctccaggaagccaggcaatgtgttgaagaccttagaccccagatctggatccaaggaaaacttgtatttccagggc

SEQ ID NO: 60 - protein, 752 aa, artificial sequence
  Synthetic construct
MERGLPLLCAVLALVLAPAGAFRNDKRGPECSQNYTTPSGVIKSPGFPEKYPNSLECTYIVFAPKMSEIILEFESFDLEPDSNPPGGMFCRYDRLEIWDGFPDVGPHIGRYCGQKTPGRIRSSSGILSMVFYTDSAIAKEGFSANYSVLQSSVSEDFKCMEALGMESGEIHSDQITASSQYSTNWSAERSRLNYPENGWTPGEDSYREWIQVDLGLLRFVTAVGTQGAISKETKKKYYVKTYKIDVSSNGEDWITIKEGNKPVLFQGNTNPTDVVVAVFPKPLITRFVRIKPATWETGISMRFEVYGCKITDYPCSGMLGMVSGLISDSQITSSNQGDRNWMPENIRLVTSRSGWALPPAPHSYINEWLQIDLGEEKIVRGIIIQGGKHRENKVFMRKFKIGYSNNGSDWKMIMDDSKRKAKSFEGNNNYDTPELRTFPALSTRFIRIYPERATHGGLGLRMELLGCEVEAPTAGPTTPNGNLVDECDDDQANCHSGTGDDFQLTGGTTVLATEKPTVIDSTIQSEFPTYGFNCEFGWGSHKTFCHWEHDNHVQLKWSVLTSKTGPIQDHTGDGNFIYSQADENQKGKVARLVSPVVYSQNSAHCMTFWYHMSGSHVGTLRVKLRYQKPEEYDQLVWMAIGHQGDHWKEGRVLLHKSLKLYQVIFEGEIGKGNLGGIAVDDISINNHISQEDCAKPADLDKKNPEIKIDETGSTPGYEGEGEGDKNISRKPGNVLKTLDPRSGSKENLYFQG

SEQ ID NO: 61 - DNA, 1437 bp, artificial sequence
  Synthetic construct
atggagagggggctgccgctcctctgcgccgtgctcgccctcgtcctcgccccggccggcgcttttcgcaacgataaaagaggtcctgaatgttcccagaactacacaacacctagtggagtgataaagtcccccggattccctgaaaaatatcccaacagccttgaatgcacttatattgtctttgcgccaaagatgtcagagattatcctggaatttgaaagctttgacctggagcctgactcaaatcctccaggggggatgttctgtcgctacgaccggctagaaatctgggatggattccctgatgttggccctcacattgggcgttactgtggacagaaaacaccaggtcgaatccgatcctcatcgggcattctctccatggttttttacaccgacagcgcgatagcaaaagaaggtttctcagcaaactacagtgtcttgcagagcagtgtctcagaagatttcaaatgtatggaagctctgggcatggaatcaggagaaattcattctgaccagatcacagcttcttcccagtatagcaccaactggtctgcagagcgctcccgcctgaactaccctgagaatgggtggactcccggagaggattcctaccgagagtggatacaggtagacttgggccttctgcgctttgtcacggctgtcgggacacagggcgccatttcaaaagaaaccaagaagaaatattatgtcaagacttacaagatcgacgttagctccaacggggaagactggatcaccataaaagaaggaaacaaacctgttctctttcagggaaacaccaaccctacagatgttgtggttgcagtattccccaaaccactgataactcgatttgtccgaatcaagcctgcaacttgggaaactggcatatctatgagatttgaagtatatggttgcaagataacagattatccttgctctggaatgttgggtatggtgtctggacttatttctgactcccagatcacatcatccaaccaaggggacagaaactggatgcctgaaaacatccgcctggtaaccagtcgctctggctgggcacttccacccgcacctcattcctacatcaatgagtggctccaaatagacctgggggaggagaagatcgtgaggggcatcatcattcagggtgggaagcaccgagagaacaaggtgttcatgaggaagttcaagatcgggtacagcaacaacggctcggactggaagatgatcatggatgacagcaaacgcaaggcgaagtcttttgagggcaacaacaactatgatacacctgagctgcggacttttccagctctctccacgcgattcatcaggatctaccccgagagagccactcatggcggactggggctcagaatggagctgctgggctgtagatctggatccaaggaaaacttgtatttccagggc

SEQ ID NO: 62 - protein, 479 aa, artificial sequence
  Synthetic construct
MERGLPLLCAVLALVLAPAGAFRNDKRGPECSQNYTTPSGVIKSPGFPEKYPNSLECTYIVFAPKMSEIILEFESFDLEPDSNPPGGMFCRYDRLEIWDGFPDVGPHIGRYCGQKTPGRIRSSSGILSMVFYTDSAIAKEGFSANYSVLQSSVSEDFKCMEALGMESGEIHSDQITASSQYSTNWSAERSRLNYPENGWTPGEDSYREWIQVDLGLLRFVTAVGTQGAISKETKKKYYVKTYKIDVSSNGEDWITIKEGNKPVLFQGNTNPTDVVVAVFPKPLITRFVRIKPATWETGISMRFEVYGCKITDYPCSGMLGMVSGLISDSQITSSNQGDRNWMPENIRLVTSRSGWALPPAPHSYINEWLQIDLGEEKIVRGIIIQGGKHRENKVFMRKFKIGYSNNGSDWKMIMDDSKRKAKSFEGNNNYDTPELRTFPALSTRFIRIYPERATHGGLGLRMELLGCRSGSKENLYFQG

SEQ ID NO: 63 - DNA, 960 bp, artificial sequence
  Synthetic construct
atggagagggggctgccgctcctctgcgccgtgctcgccctcgtcctcgccccggccggcgcttttcgcaacgataaaagaggtcctgaatgttcccagaactacacaacacctagtggagtgataaagtcccccggattccctgaaaaatatcccaacagccttgaatgcacttatattgtctttgcgccaaagatgtcagagattatcctggaatttgaaagctttgacctggagcctgactcaaatcctccaggggggatgttctgtcgctacgaccggctagaaatctgggatggattccctgatgttggccctcacattgggcgttactgtggacagaaaacaccaggtcgaatccgatcctcatcgggcattctctccatggttttttacaccgacagcgcgatagcaaaagaaggtttctcagcaaactacagtgtcttgcagagcagtgtctcagaagatttcaaatgtatggaagctctgggcatggaatcaggagaaattcattctgaccagatcacagcttcttcccagtatagcaccaactggtctgcagagcgctcccgcctgaactaccctgagaatgggtggactcccggagaggattcctaccgagagtggatacaggtagacttgggccttctgcgctttgtcacggctgtcgggacacagggcgccatttcaaaagaaaccaagaagaaatattatgtcaagacttacaagatcgacgttagctccaacggggaagactggatcaccataaaagaaggaaacaaacctgttctctttcagggaaacaccaaccctacagatgttgtggttgcagtattccccaaaccactgataactcgatttgtccgaatcaagcctgcaacttgggaaactggcatatctatgagatttgaagtatatggttgcagatctggatccaaggaaaacttgtatttccagggc

SEQ ID NO: 64 - protein, 320 aa, artificial sequence
  Synthetic construct
MERGLPLLCAVLALVLAPAGAFRNDKRGPECSQNYTTPSGVIKSPGFPEKYPNSLECTYIVFAPKMSEIILEFESFDLEPDSNPPGGMFCRYDRLEIWDGFPDVGPHIGRYCGQKTPGRIRSSSGILSMVFYTDSAIAKEGFSANYSVLQSSVSEDFKCMEALGMESGEIHSDQITASSQYSTNWSAERSRLNYPENGWTPGEDSYREWIQVDLGLLRFVTAVGTQGAISKETKKKYYVKTYKIDVSSNGEDWITIKEGNKPVLFQGNTNPTDVVVAVFPKPLITRFVRIKPATWETGISMRFEVYGCRSGSKENLYFQG

SEQ ID NO: 65 - DNA, 1797 bp, artificial sequence
  Synthetic construct
atggagagggggctgccgctcctctgcgccgtgctcgccctcgtcctcgccccggccggcgcttttcgcaacgataaaagaggtcctgaatgttcccagaactacacaacacctagtggagtgataaagtcccccggattccctgaaaaatatcccaacagccttgaatgcacttatattgtctttgcgccaaagatgtcagagattatcctggaatttgaaagctttgacctggagcctgactcaaatcctccaggggggatgttctgtcgctacgaccggctagaaatctgggatggattccctgatgttggccctcacattgggcgttactgtggacagaaaacaccaggtcgaatccgatcctcatcgggcattctctccatggttttttacaccgacagcgcgatagcaaaagaaggtttctcagcaaactacagtgtcttgcagagcagtgtctcagaagatttcaaatgtatggaagctctgggcatggaatcaggagaaattcattctgaccagatcacagcttcttcccagtatagcaccaactggtctgcagagcgctcccgcctgaactaccctgagaatgggtggactcccggagaggattcctaccgagagtggatacaggtagacttgggccttctgcgctttgtcacggctgtcgggacacagggcgccatttcaaaagaaaccaagaagaaatattatgtcaagacttacaagatcgacgttagctccaacggggaagactggatcaccataaaagaaggaaacaaacctgttctctttcagggaaacaccaaccctacagatgttgtggttgcagtattccccaaaccactgataactcgatttgtccgaatcaagcctgcaacttgggaaactggcatatctatgagatttgaagtatatggttgcaagataacagattatcctgaagtggaagcccctacagctggaccgaccactcccaacgggaacttggtggatgaatgtgatgacgaccaggccaactgccacagtggaacaggtgatgacttccagctcacaggtggcaccactgtgctggccacagaaaagcccacggtcatagacagcaccatacaatcagagtttccaacatatggttttaactgtgaatttggctggggctctcacaagaccttctgccactgggaacatgacaatcacgtgcagctcaagtggagtgtgttgaccagcaagacgggacccattcaggatcacacaggagatggcaacttcatctattcccaagctgacgaaaatcagaagggcaaagtggctcgcctggtgagccctgtggtttattcccagaactctgcccactgcatgaccttctggtatcacatgtctgggtcccacgtcggcacactcagggtcaaactgcgctaccagaagccagaggagtacgatcagctggtctggatggccattggacaccaaggtgaccactggaaggaagggcgtgtcttgctccacaagtctctgaaactttatcaggtgattttcgagggcgaaatcggaaaaggaaaccttggtgggattgctgtggatgacattagtattaataaccacatttcacaagaagattgtgcaaaaccagcagacctggataaaaagaacccagaaattaaaattgatgaaacagggagcacgccaggatacgaaggtgaaggagaaggtgacaagaacatctccaggaagccaggcaatgtgttgaagaccttagaccccagatctggatccaaggaaaacttgtatttccagggc

SEQ ID NO: 66 - protein, 599 aa, artificial sequence
  Synthetic construct
MERGLPLLCAVLALVLAPAGAFRNDKRGPECSQNYTTPSGVIKSPGFPEKYPNSLECTYIVFAPKMSEIILEFESFDLEPDSNPPGGMFCRYDRLEIWDGFPDVGPHIGRYCGQKTPGRIRSSSGILSMVFYTDSAIAKEGFSANYSVLQSSVSEDFKCMEALGMESGEIHSDQITASSQYSTNWSAERSRLNYPENGWTPGEDSYREWIQVDLGLLRFVTAVGTQGAISKETKKKYYVKTYKIDVSSNGEDWITIKEGNKPVLFQGNTNPTDVVVAVFPKPLITRFVRIKPATWETGISMRFEVYGCKITDYPEVEAPTAGPTTPNGNLVDECDDDQANCHSGTGDDFQLTGGTTVLATEKPTVIDSTIQSEFPTYGFNCEFGWGSHKTFCHWEHDNHVQLKWSVLTSKTGPIQDHTGDGNFIYSQADENQKGKVARLVSPVVYSQNSAHCMTFWYHMSGSHVGTLRVKLRYQKPEEYDQLVWMAIGHQGDHWKEGRVLLHKSLKLYQVIFEGEIGKGNLGGIAVDDISINNHISQEDCAKPADLDKKNPEIKIDETGSTPGYEGEGEGDKNISRKPGNVLKTLDPRSGSKENLYFQG

SEQ ID NO: 67 - DNA, 2604 bp, artificial sequence
  Synthetic construct
atggagagggggctgccgctcctctgcgccgtgctcgccctcgtcctcgccccggccggcgcttttcgcaacgataaatgtggcgatactataaaaattgaaagccccgggtaccttacatctcctggttatcctcattcttatcacccaagtgaaaaatgcgaatggctgattcaggctccggacccataccagagaattatgatcaacttcaaccctcacttcgatttggaggacagagactgcaagtatgactacgtggaagtcttcgatggagaaaatgaaaatggacattttaggggaaagttctgtggaaagatagcccctcctcctgttgtgtcttcagggccatttctttttatcaaatttgtctctgactacgaaacacatggtgcaggattttccatacgttatgaacttttcaagagaggtcctgaatgttcccagaactacacaacacctagtggagtgataaagtcccccggattccctgaaaaatatcccaacagccttgaatgcacttatattgtctttgcgccaaagatgtcagagattatcctggaatttgaaagctttgacctggagcctgactcaaatcctccaggggggatgttctgtcgctacgaccggctagaaatctgggatggattccctgatgttggccctcacattgggcgttactgtggacagaaaacaccaggtcgaatccgatcctcatcgggcattctctccatggttttttacaccgacagcgcgatagcaaaagaaggtttctcagcaaactacagtgtcttgcagagcagtgtctcagaagatttcaaatgtatggaagctctgggcatggaatcaggagaaattcattctgaccagatcacagcttcttcccagtatagcaccaactggtctgcagagcgctcccgcctgaactaccctgagaatgggtggactcccggagaggattcctaccgagagtggatacaggtagacttgggccttctgcgctttgtcacggctgtcgggacacagggcgccatttcaaaagaaaccaagaagaaatattatgtcaagacttacaagatcgacgttagctccaacggggaagactggatcaccataaaagaaggaaacaaacctgttctctttcagggaaacaccaaccctacagatgttgtggttgcagtattccccaaaccactgataactcgatttgtccgaatcaagcctgcaacttgggaaactggcatatctatgagatttgaagtatatggttgcaagataacagattatccttgctctggaatgttgggtatggtgtctggacttatttctgactcccagatcacatcatccaaccaaggggacagaaactggatgcctgaaaacatccgcctggtaaccagtcgctctggctgggcacttccacccgcacctcattcctacatcaatgagtggctccaaatagacctgggggaggagaagatcgtgaggggcatcatcattcagggtgggaagcaccgagagaacaaggtgttcatgaggaagttcaagatcgggtacagcaacaacggctcggactggaagatgatcatggatgacagcaaacgcaaggcgaagtcttttgagggcaacaacaactatgatacacctgagctgcggacttttccagctctctccacgcgattcatcaggatctaccccgagagagccactcatggcggactggggctcagaatggagctgctgggctgtgaagtggaagcccctacagctggaccgaccactcccaacgggaacttggtggatgaatgtgatgacgaccaggccaactgccacagtggaacaggtgatgacttccagctcacaggtggcaccactgtgctggccacagaaaagcccacggtcatagacagcaccatacaatcagagtttccaacatatggttttaactgtgaatttggctggggctctcacaagaccttctgccactgggaacatgacaatcacgtgcagctcaagtggagtgtgttgaccagcaagacgggacccattcaggatcacacaggagatggcaacttcatctattcccaagctgacgaaaatcagaagggcaaagtggctcgcctggtgagccctgtggtttattcccagaactctgcccactgcatgaccttctggtatcacatgtctgggtcccacgtcggcacactcagggtcaaactgcgctaccagaagccagaggagtacgatcagctggtctggatggccattggacaccaaggtgaccactggaaggaagggcgtgtcttgctccacaagtctctgaaactttatcaggtgattttcgagggcgaaatcggaaaaggaaaccttggtgggattgctgtggatgacattagtattaataaccacatttcacaagaagattgtgcaaaaccagcagacctggataaaaagaacccagaaattaaaattgatgaaacagggagcacgccaggatacgaaggtgaaggagaaggtgacaagaacatctccaggaagccaggcaatgtgttgaagaccttagaccccagatctggatccaaggaaaacttgtatttccagggc

SEQ ID NO: 68 - protein, 847 aa, artificial sequence
  Synthetic construct
FRNDKCGDTIKIESPGYLTSPGYPHSYHPSEKCEWLIQAPDPYQRIMINFNPHFDLEDRDCKYDYVEVFDGENENGHFRGKFCGKIAPPPVVSSGPFLFIKFVSDYETHGAGFSIRYELFKRGPECSQNYTTPSGVIKSPGFPEKYPNSLECTYIVFAPKMSEIILEFESFDLEPDSNPPGGMFCRYDRLEIWDGFPDVGPHIGRYCGQKTPGRIRSSSGILSMVFYTDSAIAKEGFSANYSVLQSSVSEDFKCMEALGMESGEIHSDQITASSQYSTNWSAERSRLNYPENGWTPGEDSYREWIQVDLGLLRFVTAVGTQGAISKETKKKYYVKTYKIDVSSNGEDWITIKEGNKPVLFQGNTNPTDVVVAVFPKPLITRFVRIKPATWETGISMRFEVYGCKITDYPCSGMLGMVSGLISDSQITSSNQGDRNWMPENIRLVTSRSGWALPPAPHSYINEWLQIDLGEEKIVRGIIIQGGKHRENKVFMRKFKIGYSNNGSDWKMIMDDSKRKAKSFEGNNNYDTPELRTFPALSTRFIRIYPERATHGGLGLRMELLGCEVEAPTAGPTTPNGNLVDECDDDQANCHSGTGDDFQLTGGTTVLATEKPTVIDSTIQSEFPTYGFNCEFGWGSHKTFCHWEHDNHVQLKWSVLTSKTGPIQDHTGDGNFIYSQADENQKGKVARLVSPVVYSQNSAHCMTFWYHMSGSHVGTLRVKLRYQKPEEYDQLVWMAIGHQGDHWKEGRVLLHKSLKLYQVIFEGEIGKGNLGGIAVDDISINNHISQEDCAKPADLDKKNPEIKIDETGSTPGYEGEGEGDKNISRKPGNVLKTLDPRSGSKENLYFQG

SEQ ID NO: 69 - DNA, 2604 bp, artificial sequence
  Synthetic construct
atggagagggggctgccgctcctctgcgccgtgctcgccctcgtcctcgccccggccggcgcttttcgcaacgataaatgtggcgatactataaaaattgaaagccccgggtaccttacatctcctggttatcctcattcttatcacccaagtgaaaaatgcgaatggctgattcaggctccggacccataccagagaattatgatcaacttcaaccctcacttcgatttggaggacagagactgcaagtatgactacgtggaagtcttcgatggagaaaatgaaaatggacattttaggggaaagttctgtggaaagatagcccctcctcctgttgtgtcttcagggccatttctttttatcaaatttgtctctgactacgaaacacatggtgcaggattttccatacgttatgaacttttcaagagaggtcctgaatgttcccagaactacacaacacctagtggagtgataaagtcccccggattccctgaaaaatatcccaacagccttgaatgcacttatattgtctttgcgccaaagatgtcagagattatcctggaatttgaaagctttgacctggagcctgactcaaatcctccaggggggatgttctgtcgctacgaccggctagaaatctgggatggattccctgatgttggccctcacattgggcgttactgtggacagaaaacaccaggtcgaatccgatcctcatcgggcattctctccatggttttttacaccgacagcgcgatagcaaaagaaggtttctcagcaaactacagtgtcttgcagagcagtgtctcagaagatttcaaatgtatggaagctctgggcatggaatcaggagaaattcattctgaccagatcacagcttcttcccaggctagcaccaactggtctgcagagcgctcccgcctgaactaccctgagaatgggtggactcccggagaggattcctaccgagagtggatacaggtagacttgggccttctgcgctttgtcacggctgtcgggacacagggcgccatttcaaaagaaaccaagaagaaatattatgtcaagacttacaagatcgacgttagctccaacggggaagactggatcaccataaaagaaggaaacaaacctgttctctttcagggaaacaccaaccctacagatgttgtggttgcagtattccccaaaccactgataactcgatttgtccgaatcaagcctgcaacttgggaaactggcatatctatgagatttgaagtatatggttgcaagataacagattatccttgctctggaatgttgggtatggtgtctggacttatttctgactcccagatcacatcatccaaccaaggggacagaaactggatgcctgaaaacatccgcctggtaaccagtcgctctggctgggcacttccacccgcacctcattcctacatcaatgagtggctccaaatagacctgggggaggagaagatcgtgaggggcatcatcattcagggtgggaagcaccgagagaacaaggtgttcatgaggaagttcaagatcgggtacagcaacaacggctcggactggaagatgatcatggatgacagcaaacgcaaggcgaagtcttttgagggcaacaacaactatgatacacctgagctgcggacttttccagctctctccacgcgattcatcaggatctaccccgagagagccactcatggcggactggggctcagaatggagctgctgggctgtgaagtggaagcccctacagctggaccgaccactcccaacgggaacttggtggatgaatgtgatgacgaccaggccaactgccacagtggaacaggtgatgacttccagctcacaggtggcaccactgtgctggccacagaaaagcccacggtcatagacagcaccatacaatcagagtttccaacatatggttttaactgtgaatttggctggggctctcacaagaccttctgccactgggaacatgacaatcacgtgcagctcaagtggagtgtgttgaccagcaagacgggacccattcaggatcacacaggagatggcaacttcatctattcccaagctgacgaaaatcagaagggcaaagtggctcgcctggtgagccctgtggtttattcccagaactctgcccactgcatgaccttctggtatcacatgtctgggtcccacgtcggcacactcagggtcaaactgcgctaccagaagccagaggagtacgatcagctggtctggatggccattggacaccaaggtgaccactggaaggaagggcgtgtcttgctccacaagtctctgaaactttatcaggtgattttcgagggcgaaatcggaaaaggaaaccttggtgggattgctgtggatgacattagtattaataaccacatttcacaagaagattgtgcaaaaccagcagacctggataaaaagaacccagaaattaaaattgatgaaacagggagcacgccaggatacgaaggtgaaggagaaggtgacaagaacatctccaggaagccaggcaatgtgttgaagaccttagaccccagatctggatccaaggaaaacttgtatttccagggc

SEQ ID NO: 70 - protein, 847 aa, artificial sequence
  Synthetic construct
FRNDKCGDTIKIESPGYLTSPGYPHSYHPSEKCEWLIQAPDPYQRIMINFNPHFDLEDRDCKYDYVEVFDGENENGHFRGKFCGKIAPPPVVSSGPFLFIKFVSDYETHGAGFSIRYELFKRGPECSQNYTTPSGVIKSPGFPEKYPNSLECTYIVFAPKMSEIILEFESFDLEPDSNPPGGMFCRYDRLEIWDGFPDVGPHIGRYCGQKTPGRIRSSSGILSMVFYTDSAIAKEGFSANYSVLQSSVSEDFKCMEALGMESGEIHSDQITASSQASTNWSAERSRLNYPENGWTPGEDSYREWIQVDLGLLRFVTAVGTQGAISKETKKKYYVKTYKIDVSSNGEDWITIKEGNKPVLFQGNTNPTDVVVAVFPKPLITRFVRIKPATWETGISMRFEVYGCKITDYPCSGMLGMVSGLISDSQITSSNQGDRNWMPENIRLVTSRSGWALPPAPHSYINEWLQIDLGEEKIVRGIIIQGGKHRENKVFMRKFKIGYSNNGSDWKMIMDDSKRKAKSFEGNNNYDTPELRTFPALSTRFIRIYPERATHGGLGLRMELLGCEVEAPTAGPTTPNGNLVDECDDDQANCHSGTGDDFQLTGGTTVLATEKPTVIDSTIQSEFPTYGFNCEFGWGSHKTFCHWEHDNHVQLKWSVLTSKTGPIQDHTGDGNFIYSQADENQKGKVARLVSPVVYSQNSAHCMTFWYHMSGSHVGTLRVKLRYQKPEEYDQLVWMAIGHQGDHWKEGRVLLHKSLKLYQVIFEGEIGKGNLGGIAVDDISINNHISQEDCAKPADLDKKNPEIKIDETGSTPGYEGEGEGDKNISRKPGNVLKTLDPRSGSKENLYFQG

SEQ ID NO: 71 - DNA, 2604 bp, artificial sequence
  Synthetic construct
atggagagggggctgccgctcctctgcgccgtgctcgccctcgtcctcgccccggccggcgcttttcgcaacgataaatgtggcgatactataaaaattgaaagccccgggtaccttacatctcctggttatcctcattcttatcacccaagtgaaaaatgcgaatggctgattcaggctccggacccataccagagaattatgatcaacttcaaccctcacttcgatttggaggacagagactgcaagtatgactacgtggaagtcttcgatggagaaaatgaaaatggacattttaggggaaagttctgtggaaagatagcccctcctcctgttgtgtcttcagggccatttctttttatcaaatttgtctctgactacgaaacacatggtgcaggattttccatacgttatgaacttttcaagagaggtcctgaatgttcccagaactacacaacacctagtggagtgataaagtcccccggattccctgaaaaatatcccaacagccttgaatgcacttatattgtctttgcgccaaagatgtcagagattatcctggaatttgaaagctttgacctggagcctgactcaaatcctccaggggggatgttctgtcgctacgaccggctagaaatctgggatggattccctgatgttggccctcacattgggcgttactgtggacagaaaacaccaggtcgaatccgatcctcatcgggcattctctccatggttttttacaccgacagcgcgatagcaaaagaaggtttctcagcaaactacagtgtcttgcagagcagtgtctcagaagatttcaaatgtatggaagctctgggcatggaatcaggagaaattcattctgaccagatcacagcttcttcccagtatagcaccaactggtctgcagagcgctcccgcctgaactaccctgagaatgggtggactcccggaaagaagtcctaccgagagtggatacaggtagacttgggccttctgcgctttgtcacggctgtcgggacacagggcgccatttcaaaagaaaccaagaagaaatattatgtcaagacttacaagatcgacgttagctccaacggggaagactggatcaccataaaagaaggaaacaaacctgttctctttcagggaaacaccaaccctacagatgttgtggttgcagtattccccaaaccactgataactcgatttgtccgaatcaagcctgcaacttgggaaactggcatatctatgagatttgaagtatatggttgcaagataacagattatccttgctctggaatgttgggtatggtgtctggacttatttctgactcccagatcacatcatccaaccaaggggacagaaactggatgcctgaaaacatccgcctggtaaccagtcgctctggctgggcacttccacccgcacctcattcctacatcaatgagtggctccaaatagacctgggggaggagaagatcgtgaggggcatcatcattcagggtgggaagcaccgagagaacaaggtgttcatgaggaagttcaagatcgggtacagcaacaacggctcggactggaagatgatcatggatgacagcaaacgcaaggcgaagtcttttgagggcaacaacaactatgatacacctgagctgcggacttttccagctctctccacgcgattcatcaggatctaccccgagagagccactcatggcggactggggctcagaatggagctgctgggctgtgaagtggaagcccctacagctggaccgaccactcccaacgggaacttggtggatgaatgtgatgacgaccaggccaactgccacagtggaacaggtgatgacttccagctcacaggtggcaccactgtgctggccacagaaaagcccacggtcatagacagcaccatacaatcagagtttccaacatatggttttaactgtgaatttggctggggctctcacaagaccttctgccactgggaacatgacaatcacgtgcagctcaagtggagtgtgttgaccagcaagacgggacccattcaggatcacacaggagatggcaacttcatctattcccaagctgacgaaaatcagaagggcaaagtggctcgcctggtgagccctgtggtttattcccagaactctgcccactgcatgaccttctggtatcacatgtctgggtcccacgtcggcacactcagggtcaaactgcgctaccagaagccagaggagtacgatcagctggtctggatggccattggacaccaaggtgaccactggaaggaagggcgtgtcttgctccacaagtctctgaaactttatcaggtgattttcgagggcgaaatcggaaaaggaaaccttggtgggattgctgtggatgacattagtattaataaccacatttcacaagaagattgtgcaaaaccagcagacctggataaaaagaacccagaaattaaaattgatgaaacagggagcacgccaggatacgaaggtgaaggagaaggtgacaagaacatctccaggaagccaggcaatgtgttgaagaccttagaccccagatctggatccaaggaaaacttgtatttccagggc

SEQ ID NO: 72 - protein, 847 aa, artificial sequence
  Synthetic construct
FRNDKCGDTIKIESPGYLTSPGYPHSYHPSEKCEWLIQAPDPYQRIMINFNPHFDLEDRDCKYDYVEVFDGENENGHFRGKFCGKIAPPPVVSSGPFLFIKFVSDYETHGAGFSIRYELFKRGPECSQNYTTPSGVIKSPGFPEKYPNSLECTYIVFAPKMSEIILEFESFDLEPDSNPPGGMFCRYDRLEIWDGFPDVGPHIGRYCGQKTPGRIRSSSGILSMVFYTDSAIAKEGFSANYSVLQSSVSEDFKCMEALGMESGEIHSDQITASSQYSTNWSAERSRLNYPENGWTPGKKSYREWIQVDLGLLRFVTAVGTQGAISKETKKKYYVKTYKIDVSSNGEDWITIKEGNKPVLFQGNTNPTDVVVAVFPKPLITRFVRIKPATWETGISMRFEVYGCKITDYPCSGMLGMVSGLISDSQITSSNQGDRNWMPENIRLVTSRSGWALPPAPHSYINEWLQIDLGEEKIVRGIIIQGGKHRENKVFMRKFKIGYSNNGSDWKMIMDDSKRKAKSFEGNNNYDTPELRTFPALSTRFIRIYPERATHGGLGLRMELLGCEVEAPTAGPTTPNGNLVDECDDDQANCHSGTGDDFQLTGGTTVLATEKPTVIDSTIQSEFPTYGFNCEFGWGSHKTFCHWEHDNHVQLKWSVLTSKTGPIQDHTGDGNFIYSQADENQKGKVARLVSPVVYSQNSAHCMTFWYHMSGSHVGTLRVKLRYQKPEEYDQLVWMAIGHQGDHWKEGRVLLHKSLKLYQVIFEGEIGKGNLGGIAVDDISINNHISQEDCAKPADLDKKNPEIKIDETGSTPGYEGEGEGDKNISRKPGNVLKTLDPRSGSKENLYFQG

SEQ ID NO: 73 - DNA, 2604 bp, artificial sequence
  Synthetic construct
atggagagggggctgccgctcctctgcgccgtgctcgccctcgtcctcgccccggccggcgcttttcgcaacgataaatgtggcgatactataaaaattgaaagccccgggtaccttacatctcctggttatcctcattcttatcacccaagtgaaaaatgcgaatggctgattcaggctccggacccataccagagaattatgatcaacttcaaccctcacttcgatttggaggacagagactgcaagtatgactacgtggaagtcttcgatggagaaaatgaaaatggacattttaggggaaagttctgtggaaagatagcccctcctcctgttgtgtcttcagggccatttctttttatcaaatttgtctctgactacgaaacacatggtgcaggattttccatacgttatgaacttttcaagagaggtcctgaatgttcccagaactacacaacacctagtggagtgataaagtcccccggattccctgaaaaatatcccaacagccttgaatgcacttatattgtctttgcgccaaagatgtcagagattatcctggaatttgaaagctttgacctggagcctgactcaaatcctccaggggggatgttctgtcgctacgaccggctagaaatctgggatggattccctgatgttggccctcacattgggcgttactgtggacagaaaacaccaggtcgaatccgatcctcatcgggcattctctccatggttttttacaccgacagcgcgatagcaaaagaaggtttctcagcaaactacagtgtcttgcagagcagtgtctcagaagatttcaaatgtatggaagctctgggcatggaatcaggagaaattcattctgaccagatcacagcttcttcccagtatagcaccaactggtctgcagagcgctcccgcctgaactaccctgagaatgggtggactcccggagaggattcctaccgagagtggatacaggtagacttgggccttctgcgctttgtcacggctgtcgggacacagggcgccattgccaaaaagaccaagaagaaatattatgtcaagacttacaagatcgacgttagctccaacggggaagactggatcaccataaaagaaggaaacaaacctgttctctttcagggaaacaccaaccctacagatgttgtggttgcagtattccccaaaccactgataactcgatttgtccgaatcaagcctgcaacttgggaaactggcatatctatgagatttgaagtatatggttgcaagataacagattatccttgctctggaatgttgggtatggtgtctggacttatttctgactcccagatcacatcatccaaccaaggggacagaaactggatgcctgaaaacatccgcctggtaaccagtcgctctggctgggcacttccacccgcacctcattcctacatcaatgagtggctccaaatagacctgggggaggagaagatcgtgaggggcatcatcattcagggtgggaagcaccgagagaacaaggtgttcatgaggaagttcaagatcgggtacagcaacaacggctcggactggaagatgatcatggatgacagcaaacgcaaggcgaagtcttttgagggcaacaacaactatgatacacctgagctgcggacttttccagctctctccacgcgattcatcaggatctaccccgagagagccactcatggcggactggggctcagaatggagctgctgggctgtgaagtggaagcccctacagctggaccgaccactcccaacgggaacttggtggatgaatgtgatgacgaccaggccaactgccacagtggaacaggtgatgacttccagctcacaggtggcaccactgtgctggccacagaaaagcccacggtcatagacagcaccatacaatcagagtttccaacatatggttttaactgtgaatttggctggggctctcacaagaccttctgccactgggaacatgacaatcacgtgcagctcaagtggagtgtgttgaccagcaagacgggacccattcaggatcacacaggagatggcaacttcatctattcccaagctgacgaaaatcagaagggcaaagtggctcgcctggtgagccctgtggtttattcccagaactctgcccactgcatgaccttctggtatcacatgtctgggtcccacgtcggcacactcagggtcaaactgcgctaccagaagccagaggagtacgatcagctggtctggatggccattggacaccaaggtgaccactggaaggaagggcgtgtcttgctccacaagtctctgaaactttatcaggtgattttcgagggcgaaatcggaaaaggaaaccttggtgggattgctgtggatgacattagtattaataaccacatttcacaagaagattgtgcaaaaccagcagacctggataaaaagaacccagaaattaaaattgatgaaacagggagcacgccaggatacgaaggtgaaggagaaggtgacaagaacatctccaggaagccaggcaatgtgttgaagaccttagaccccagatctggatccaaggaaaacttgtatttccagggc

SEQ ID NO: 74 - protein, 847 aa, artificial sequence
  Synthetic construct
FRNDKCGDTIKIESPGYLTSPGYPHSYHPSEKCEWLIQAPDPYQRIMINFNPHFDLEDRDCKYDYVEVFDGENENGHFRGKFCGKIAPPPVVSSGPFLFIKFVSDYETHGAGFSIRYELFKRGPECSQNYTTPSGVIKSPGFPEKYPNSLECTYIVFAPKMSEIILEFESFDLEPDSNPPGGMFCRYDRLEIWDGFPDVGPHIGRYCGQKTPGRIRSSSGILSMVFYTDSAIAKEGFSANYSVLQSSVSEDFKCMEALGMESGEIHSDQITASSQYSTNWSAERSRLNYPENGWTPGEDSYREWIQVDLGLLRFVTAVGTQGAIAKKTKKKYYVKTYKIDVSSNGEDWITIKEGNKPVLFQGNTNPTDVVVAVFPKPLITRFVRIKPATWETGISMRFEVYGCKITDYPCSGMLGMVSGLISDSQITSSNQGDRNWMPENIRLVTSRSGWALPPAPHSYINEWLQIDLGEEKIVRGIIIQGGKHRENKVFMRKFKIGYSNNGSDWKMIMDDSKRKAKSFEGNNNYDTPELRTFPALSTRFIRIYPERATHGGLGLRMELLGCEVEAPTAGPTTPNGNLVDECDDDQANCHSGTGDDFQLTGGTTVLATEKPTVIDSTIQSEFPTYGFNCEFGWGSHKTFCHWEHDNHVQLKWSVLTSKTGPIQDHTGDGNFIYSQADENQKGKVARLVSPVVYSQNSAHCMTFWYHMSGSHVGTLRVKLRYQKPEEYDQLVWMAIGHQGDHWKEGRVLLHKSLKLYQVIFEGEIGKGNLGGIAVDDISINNHISQEDCAKPADLDKKNPEIKIDETGSTPGYEGEGEGDKNISRKPGNVLKTLDPRSGSKENLYFQG

SEQ ID NO: 75 - DNA, 2604 bp, artificial sequence
  Synthetic construct
atggagagggggctgccgctcctctgcgccgtgctcgccctcgtcctcgccccggccggcgcttttcgcaacgataaatgtggcgatactataaaaattgaaagccccgggtaccttacatctcctggttatcctcattcttatcacccaagtgaaaaatgcgaatggctgattcaggctccggacccataccagagaattatgatcaacttcaaccctcacttcgatttggaggacagagactgcaagtatgactacgtggaagtcttcgatggagaaaatgaaaatggacattttaggggaaagttctgtggaaagatagcccctcctcctgttgtgtcttcagggccatttctttttatcaaatttgtctctgactacgaaacacatggtgcaggattttccatacgttatgaacttttcaagagaggtcctgaatgttcccagaactacacaacacctagtggagtgataaagtcccccggattccctgaaaaatatcccaacagccttgaatgcacttatattgtctttgcgccaaagatgtcagagattatcctggaatttgaaagctttgacctggagcctgactcaaatcctccaggggggatgttctgtcgctacgaccggctagaaatctgggatggattccctgatgttggccctcacattgggcgttactgtggacagaaaacaccaggtcgaatccgatcctcatcgggcattctctccatggttttttacaccgacagcgcgatagcaaaagaaggtttctcagcaaactacagtgtcttgcagagcagtgtctcagaagatttcaaatgtatggaagctctgggcatggaatcaggagaaattcattctgaccagatcacagcttcttcccagtatagcaccaactggtctgcagagcgctcccgcctgaactaccctgagaatgggtggactcccggagagaagtcctaccgagagtggatacaggtagacttgggccttctgcgctttgtcacggctgtcgggacacagggcgccatttcaaaagaaaccaagaagaaatattatgtcaagacttacaagatcgacgttagctccaacggggaagactggatcaccataaaagaaggaaacaaacctgttctctttcagggaaacaccaaccctacagatgttgtggttgcagtattccccaaaccactgataactcgatttgtccgaatcaagcctgcaacttgggaaactggcatatctatgagatttgaagtatatggttgcaagataacagattatccttgctctggaatgttgggtatggtgtctggacttatttctgactcccagatcacatcatccaaccaaggggacagaaactggatgcctgaaaacatccgcctggtaaccagtcgctctggctgggcacttccacccgcacctcattcctacatcaatgagtggctccaaatagacctgggggaggagaagatcgtgaggggcatcatcattcagggtgggaagcaccgagagaacaaggtgttcatgaggaagttcaagatcgggtacagcaacaacggctcggactggaagatgatcatggatgacagcaaacgcaaggcgaagtcttttgagggcaacaacaactatgatacacctgagctgcggacttttccagctctctccacgcgattcatcaggatctaccccgagagagccactcatggcggactggggctcagaatggagctgctgggctgtgaagtggaagcccctacagctggaccgaccactcccaacgggaacttggtggatgaatgtgatgacgaccaggccaactgccacagtggaacaggtgatgacttccagctcacaggtggcaccactgtgctggccacagaaaagcccacggtcatagacagcaccatacaatcagagtttccaacatatggttttaactgtgaatttggctggggctctcacaagaccttctgccactgggaacatgacaatcacgtgcagctcaagtggagtgtgttgaccagcaagacgggacccattcaggatcacacaggagatggcaacttcatctattcccaagctgacgaaaatcagaagggcaaagtggctcgcctggtgagccctgtggtttattcccagaactctgcccactgcatgaccttctggtatcacatgtctgggtcccacgtcggcacactcagggtcaaactgcgctaccagaagccagaggagtacgatcagctggtctggatggccattggacaccaaggtgaccactggaaggaagggcgtgtcttgctccacaagtctctgaaactttatcaggtgattttcgagggcgaaatcggaaaaggaaaccttggtgggattgctgtggatgacattagtattaataaccacatttcacaagaagattgtgcaaaaccagcagacctggataaaaagaacccagaaattaaaattgatgaaacagggagcacgccaggatacgaaggtgaaggagaaggtgacaagaacatctccaggaagccaggcaatgtgttgaagaccttagaccccagatctggatccaaggaaaacttgtatttccagggc

SEQ ID NO: 76 - protein, 847 aa, artificial sequence
  Synthetic construct
FRNDKCGDTIKIESPGYLTSPGYPHSYHPSEKCEWLIQAPDPYQRIMINFNPHFDLEDRDCKYDYVEVFDGENENGHFRGKFCGKIAPPPVVSSGPFLFIKFVSDYETHGAGFSIRYELFKRGPECSQNYTTPSGVIKSPGFPEKYPNSLECTYIVFAPKMSEIILEFESFDLEPDSNPPGGMFCRYDRLEIWDGFPDVGPHIGRYCGQKTPGRIRSSSGILSMVFYTDSAIAKEGFSANYSVLQSSVSEDFKCMEALGMESGEIHSDQITASSQYSTNWSAERSRLNYPENGWTPGEKSYREWIQVDLGLLRFVTAVGTQGAISKETKKKYYVKTYKIDVSSNGEDWITIKEGNKPVLFQGNTNPTDVVVAVFPKPLITRFVRIKPATWETGISMRFEVYGCKITDYPCSGMLGMVSGLISDSQITSSNQGDRNWMPENIRLVTSRSGWALPPAPHSYINEWLQIDLGEEKIVRGIIIQGGKHRENKVFMRKFKIGYSNNGSDWKMIMDDSKRKAKSFEGNNNYDTPELRTFPALSTRFIRIYPERATHGGLGLRMELLGCEVEAPTAGPTTPNGNLVDECDDDQANCHSGTGDDFQLTGGTTVLATEKPTVIDSTIQSEFPTYGFNCEFGWGSHKTFCHWEHDNHVQLKWSVLTSKTGPIQDHTGDGNFIYSQADENQKGKVARLVSPVVYSQNSAHCMTFWYHMSGSHVGTLRVKLRYQKPEEYDQLVWMAIGHQGDHWKEGRVLLHKSLKLYQVIFEGEIGKGNLGGIAVDDISINNHISQEDCAKPADLDKKNPEIKIDETGSTPGYEGEGEGDKNISRKPGNVLKTLDPRSGSKENLYFQG

SEQ ID NO: 77 - DNA, 1785 bp, artificial sequence
  Synthetic construct
atggagagggggctgccgctcctctgcgccgtgctcgccctcgtcctcgccccggccggcgcttttcgcaacgataaatgtggcgatactataaaaattgaaagccccgggtaccttacatctcctggttatcctcattcttatcacccaagtgaaaaatgcgaatggctgattcaggctccggacccataccagagaattatgatcaacttcaaccctcacttcgatttggaggacagagactgcaagtatgactacgtggaagtcttcgatggagaaaatgaaaatggacattttaggggaaagttctgtggaaagatagcccctcctcctgttgtgtcttcagggccatttctttttatcaaatttgtctctgactacgaaacacatggtgcaggattttccatacgttatgaacttttcaagagaggtcctgaatgttcccagaactacacaacacctagtggagtgataaagtcccccggattccctgaaaaatatcccaacagccttgaatgcacttatattgtctttgcgccaaagatgtcagagattatcctggaatttgaaagctttgacctggagcctgactcaaatcctccaggggggatgttctgtcgctacgaccggctagaaatctgggatggattccctgatgttggccctcacattgggcgttactgtggacagaaaacaccaggtcgaatccgatcctcatcgggcattctctccatggttttttacaccgacagcgcgatagcaaaagaaggtttctcagcaaactacagtgtcttgcagagcagtgtctcagaagatttcaaatgtatggaagctctgggcatggaatcaggagaaattcattctgaccagatcacagcttcttcccagtatagcaccaactggtctgcagagcgctcccgcctgaactaccctgagaatgggtggactcccggagaggattcctaccgagagtggatacaggtagacttgggccttctgcgctttgtcacggctgtcgggacacagggcgccatttcaaaagaaaccaagaagaaatattatgtcaagacttacaagatcgacgttagctccaacggggaagactggatcaccataaaagaaggaaacaaacctgttctctttcagggaaacaccaaccctacagatgttgtggttgcagtattccccaaaccactgataactcgatttgtccgaatcaagcctgcaacttgggaaactggcatatctatgagatttgaagtatatggttgcaagataacagattatccttgctctggaatgttgggtatggtgtctggacttatttctgactcccagatcacatcatccaaccaaggggacagaaactggatgcctgaaaacatccgcctggtaaccagtcgctctggctgggcacttccacccgcacctcattcctacatcaatgagtggctccaaatagacctgggggaggagaagatcgtgaggggcatcatcattcagggtgggaagcaccgagagaacaaggtgttcatgaggaagttcaagatcgggtacagcaacaacggctcggactggaagatgatcatggatgacagcaaacgcaaggcgaagtcttttgagggcaacaacaactatgatacacctgagctgcggacttttccagctctctccacgcgattcatcaggatctaccccgagagagccactcatggcggactggggctcagaatggagctgctgggctgtagatctggatccaaggaaaacttgtatttccagggc

SEQ ID NO: 78 - protein, 574 aa, artificial sequence
  Synthetic construct
FRNDKCGDTIKIESPGYLTSPGYPHSYHPSEKCEWLIQAPDPYQRIMINFNPHFDLEDRDCKYDYVEVFDGENENGHFRGKFCGKIAPPPVVSSGPFLFIKFVSDYETHGAGFSIRYELFKRGPECSQNYTTPSGVIKSPGFPEKYPNSLECTYIVFAPKMSEIILEFESFDLEPDSNPPGGMFCRYDRLEIWDGFPDVGPHIGRYCGQKTPGRIRSSSGILSMVFYTDSAIAKEGFSANYSVLQSSVSEDFKCMEALGMESGEIHSDQITASSQYSTNWSAERSRLNYPENGWTPGEDSYREWIQVDLGLLRFVTAVGTQGAISKETKKKYYVKTYKIDVSSNGEDWITIKEGNKPVLFQGNTNPTDVVVAVFPKPLITRFVRIKPATWETGISMRFEVYGCKITDYPCSGMLGMVSGLISDSQITSSNQGDRNWMPENIRLVTSRSGWALPPAPHSYINEWLQIDLGEEKIVRGIIIQGGKHRENKVFMRKFKIGYSNNGSDWKMIMDDSKRKAKSFEGNNNYDTPELRTFPALSTRFIRIYPERATHGGLGLRMELLGCRSGSKENLYFQG

SEQ ID NO: 79 - DNA, 1785 bp, artificial sequence
  Synthetic construct
atggagagggggctgccgctcctctgcgccgtgctcgccctcgtcctcgccccggccggcgcttttcgcaacgataaatgtggcgatactataaaaattgaaagccccgggtaccttacatctcctggttatcctcattcttatcacccaagtgaaaaatgcgaatggctgattcaggctccggacccataccagagaattatgatcaacttcaaccctcacttcgatttggaggacagagactgcaagtatgactacgtggaagtcttcgatggagaaaatgaaaatggacattttaggggaaagttctgtggaaagatagcccctcctcctgttgtgtcttcagggccatttctttttatcaaatttgtctctgactacgaaacacatggtgcaggattttccatacgttatgaacttttcaagagaggtcctgaatgttcccagaactacacaacacctagtggagtgataaagtcccccggattccctgaaaaatatcccaacagccttgaatgcacttatattgtctttgcgccaaagatgtcagagattatcctggaatttgaaagctttgacctggagcctgactcaaatcctccaggggggatgttctgtcgctacgaccggctagaaatctgggatggattccctgatgttggccctcacattgggcgttactgtggacagaaaacaccaggtcgaatccgatcctcatcgggcattctctccatggttttttacaccgacagcgcgatagcaaaagaaggtttctcagcaaactacagtgtcttgcagagcagtgtctcagaagatttcaaatgtatggaagctctgggcatggaatcaggagaaattcattctgaccagatcacagcttcttcccaggctagcaccaactggtctgcagagcgctcccgcctgaactaccctgagaatgggtggactcccggagaggattcctaccgagagtggatacaggtagacttgggccttctgcgctttgtcacggctgtcgggacacagggcgccatttcaaaagaaaccaagaagaaatattatgtcaagacttacaagatcgacgttagctccaacggggaagactggatcaccataaaagaaggaaacaaacctgttctctttcagggaaacaccaaccctacagatgttgtggttgcagtattccccaaaccactgataactcgatttgtccgaatcaagcctgcaacttgggaaactggcatatctatgagatttgaagtatatggttgcaagataacagattatccttgctctggaatgttgggtatggtgtctggacttatttctgactcccagatcacatcatccaaccaaggggacagaaactggatgcctgaaaacatccgcctggtaaccagtcgctctggctgggcacttccacccgcacctcattcctacatcaatgagtggctccaaatagacctgggggaggagaagatcgtgaggggcatcatcattcagggtgggaagcaccgagagaacaaggtgttcatgaggaagttcaagatcgggtacagcaacaacggctcggactggaagatgatcatggatgacagcaaacgcaaggcgaagtcttttgagggcaacaacaactatgatacacctgagctgcggacttttccagctctctccacgcgattcatcaggatctaccccgagagagccactcatggcggactggggctcagaatggagctgctgggctgtagatctggatccaaggaaaacttgtatttccagggc

SEQ ID NO: 80 - protein, 574 aa, artificial sequence
  Synthetic construct
FRNDKCGDTIKIESPGYLTSPGYPHSYHPSEKCEWLIQAPDPYQRIMINFNPHFDLEDRDCKYDYVEVFDGENENGHFRGKFCGKIAPPPVVSSGPFLFIKFVSDYETHGAGFSIRYELFKRGPECSQNYTTPSGVIKSPGFPEKYPNSLECTYIVFAPKMSEIILEFESFDLEPDSNPPGGMFCRYDRLEIWDGFPDVGPHIGRYCGQKTPGRIRSSSGILSMVFYTDSAIAKEGFSANYSVLQSSVSEDFKCMEALGMESGEIHSDQITASSQASTNWSAERSRLNYPENGWTPGEDSYREWIQVDLGLLRFVTAVGTQGAISKETKKKYYVKTYKIDVSSNGEDWITIKEGNKPVLFQGNTNPTDVVVAVFPKPLITRFVRIKPATWETGISMRFEVYGCKITDYPCSGMLGMVSGLISDSQITSSNQGDRNWMPENIRLVTSRSGWALPPAPHSYINEWLQIDLGEEKIVRGIIIQGGKHRENKVFMRKFKIGYSNNGSDWKMIMDDSKRKAKSFEGNNNYDTPELRTFPALSTRFIRIYPERATHGGLGLRMELLGCRSGSKENLYFQG

SEQ ID NO: 81 - DNA, 1308 bp, artificial sequence
  Synthetic construct
atggagagggggctgccgctcctctgcgccgtgctcgccctcgtcctcgccccggccggcgcttttcgcaacgataaatgtggcgatactataaaaattgaaagccccgggtaccttacatctcctggttatcctcattcttatcacccaagtgaaaaatgcgaatggctgattcaggctccggacccataccagagaattatgatcaacttcaaccctcacttcgatttggaggacagagactgcaagtatgactacgtggaagtcttcgatggagaaaatgaaaatggacattttaggggaaagttctgtggaaagatagcccctcctcctgttgtgtcttcagggccatttctttttatcaaatttgtctctgactacgaaacacatggtgcaggattttccatacgttatgaacttttcaagagaggtcctgaatgttcccagaactacacaacacctagtggagtgataaagtcccccggattccctgaaaaatatcccaacagccttgaatgcacttatattgtctttgcgccaaagatgtcagagattatcctggaatttgaaagctttgacctggagcctgactcaaatcctccaggggggatgttctgtcgctacgaccggctagaaatctgggatggattccctgatgttggccctcacattgggcgttactgtggacagaaaacaccaggtcgaatccgatcctcatcgggcattctctccatggttttttacaccgacagcgcgatagcaaaagaaggtttctcagcaaactacagtgtcttgcagagcagtgtctcagaagatttcaaatgtatggaagctctgggcatggaatcaggagaaattcattctgaccagatcacagcttcttcccagtatagcaccaactggtctgcagagcgctcccgcctgaactaccctgagaatgggtggactcccggagaggattcctaccgagagtggatacaggtagacttgggccttctgcgctttgtcacggctgtcgggacacagggcgccatttcaaaagaaaccaagaagaaatattatgtcaagacttacaagatcgacgttagctccaacggggaagactggatcaccataaaagaaggaaacaaacctgttctctttcagggaaacaccaaccctacagatgttgtggttgcagtattccccaaaccactgataactcgatttgtccgaatcaagcctgcaacttgggaaactggcatatctatgagatttgaagtatatggttgcagatctggatccaaggaaaacttgtatttccagggc

SEQ ID NO: 82 - protein, 415 aa, artificial sequence
  Synthetic construct
FRNDKCGDTIKIESPGYLTSPGYPHSYHPSEKCEWLIQAPDPYQRIMINFNPHFDLEDRDCKYDYVEVFDGENENGHFRGKFCGKIAPPPVVSSGPFLFIKFVSDYETHGAGFSIRYELFKRGPECSQNYTTPSGVIKSPGFPEKYPNSLECTYIVFAPKMSEIILEFESFDLEPDSNPPGGMFCRYDRLEIWDGFPDVGPHIGRYCGQKTPGRIRSSSGILSMVFYTDSAIAKEGFSANYSVLQSSVSEDFKCMEALGMESGEIHSDQITASSQYSTNWSAERSRLNYPENGWTPGEDSYREWIQVDLGLLRFVTAVGTQGAISKETKKKYYVKTYKIDVSSNGEDWITIKEGNKPVLFQGNTNPTDVVVAVFPKPLITRFVRIKPATWETGISMRFEVYGCRSGSKENLYFQG

SEQ ID NO: 83 - DNA, 1308 bp, artificial sequence
  Synthetic construct
atggagagggggctgccgctcctctgcgccgtgctcgccctcgtcctcgccccggccggcgcttttcgcaacgataaatgtggcgatactataaaaattgaaagccccgggtaccttacatctcctggttatcctcattcttatcacccaagtgaaaaatgcgaatggctgattcaggctccggacccataccagagaattatgatcaacttcaaccctcacttcgatttggaggacagagactgcaagtatgactacgtggaagtcttcgatggagaaaatgaaaatggacattttaggggaaagttctgtggaaagatagcccctcctcctgttgtgtcttcagggccatttctttttatcaaatttgtctctgactacgaaacacatggtgcaggattttccatacgttatgaacttttcaagagaggtcctgaatgttcccagaactacacaacacctagtggagtgataaagtcccccggattccctgaaaaatatcccaacagccttgaatgcacttatattgtctttgcgccaaagatgtcagagattatcctggaatttgaaagctttgacctggagcctgactcaaatcctccaggggggatgttctgtcgctacgaccggctagaaatctgggatggattccctgatgttggccctcacattgggcgttactgtggacagaaaacaccaggtcgaatccgatcctcatcgggcattctctccatggttttttacaccgacagcgcgatagcaaaagaaggtttctcagcaaactacagtgtcttgcagagcagtgtctcagaagatttcaaatgtatggaagctctgggcatggaatcaggagaaattcattctgaccagatcacagcttcttcccaggctagcaccaactggtctgcagagcgctcccgcctgaactaccctgagaatgggtggactcccggagaggattcctaccgagagtggatacaggtagacttgggccttctgcgctttgtcacggctgtcgggacacagggcgccatttcaaaagaaaccaagaagaaatattatgtcaagacttacaagatcgacgttagctccaacggggaagactggatcaccataaaagaaggaaacaaacctgttctctttcagggaaacaccaaccctacagatgttgtggttgcagtattccccaaaccactgataactcgatttgtccgaatcaagcctgcaacttgggaaactggcatatctatgagatttgaagtatatggttgcagatctggatccaaggaaaacttgtatttccagggc

SEQ ID NO: 84 - protein, 415 aa, artificial sequence
  Synthetic construct
FRNDKCGDTIKIESPGYLTSPGYPHSYHPSEKCEWLIQAPDPYQRIMINFNPHFDLEDRDCKYDYVEVFDGENENGHFRGKFCGKIAPPPVVSSGPFLFIKFVSDYETHGAGFSIRYELFKRGPECSQNYTTPSGVIKSPGFPEKYPNSLECTYIVFAPKMSEIILEFESFDLEPDSNPPGGMFCRYDRLEIWDGFPDVGPHIGRYCGQKTPGRIRSSSGILSMVFYTDSAIAKEGFSANYSVLQSSVSEDFKCMEALGMESGEIHSDQITASSQASTNWSAERSRLNYPENGWTPGEDSYREWIQVDLGLLRFVTAVGTQGAISKETKKKYYVKTYKIDVSSNGEDWITIKEGNKPVLFQGNTNPTDVVVAVFPKPLITRFVRIKPATWETGISMRFEVYGCRSGSKENLYFQG

SEQ ID NO: 85 - DNA, 831 bp, artificial sequence
  Synthetic construct
atggagagggggctgccgctcctctgcgccgtgctcgccctcgtcctcgccccggccggcgcttttcgcaacgataaatgtggcgatactataaaaattgaaagccccgggtaccttacatctcctggttatcctcattcttatcacccaagtgaaaaatgcgaatggctgattcaggctccggacccataccagagaattatgatcaacttcaaccctcacttcgatttggaggacagagactgcaagtatgactacgtggaagtcttcgatggagaaaatgaaaatggacattttaggggaaagttctgtggaaagatagcccctcctcctgttgtgtcttcagggccatttctttttatcaaatttgtctctgactacgaaacacatggtgcaggattttccatacgttatgaacttttcaagagaggtcctgaatgttcccagaactacacaacacctagtggagtgataaagtcccccggattccctgaaaaatatcccaacagccttgaatgcacttatattgtctttgcgccaaagatgtcagagattatcctggaatttgaaagctttgacctggagcctgactcaaatcctccaggggggatgttctgtcgctacgaccggctagaaatctgggatggattccctgatgttggccctcacattgggcgttactgtggacagaaaacaccaggtcgaatccgatcctcatcgggcattctctccatggttttttacaccgacagcgcgatagcaaaagaaggtttctcagcaaactacagtgtcttgagatctggatccaaggaaaacttgtatttccagggc

SEQ ID NO: 86 - protein, 256 aa, artificial sequence
  Synthetic construct
FRNDKCGDTIKIESPGYLTSPGYPHSYHPSEKCEWLIQAPDPYQRIMINFNPHFDLEDRDCKYDYVEVFDGENENGHFRGKFCGKIAPPPVVSSGPFLFIKFVSDYETHGAGFSIRYELFKRGPECSQNYTTPSGVIKSPGFPEKYPNSLECTYIVFAPKMSEIILEFESFDLEPDSNPPGGMFCRYDRLEIWDGFPDVGPHIGRYCGQKTPGRIRSSSGILSMVFYTDSAIAKEGFSANYSVLRSGSKENLYFQG

SEQ ID NO: 87 - DNA, 2145 bp, artificial sequence
  Synthetic construct
atggagagggggctgccgctcctctgcgccgtgctcgccctcgtcctcgccccggccggcgcttttcgcaacgataaatgtggcgatactataaaaattgaaagccccgggtaccttacatctcctggttatcctcattcttatcacccaagtgaaaaatgcgaatggctgattcaggctccggacccataccagagaattatgatcaacttcaaccctcacttcgatttggaggacagagactgcaagtatgactacgtggaagtcttcgatggagaaaatgaaaatggacattttaggggaaagttctgtggaaagatagcccctcctcctgttgtgtcttcagggccatttctttttatcaaatttgtctctgactacgaaacacatggtgcaggattttccatacgttatgaacttttcaagagaggtcctgaatgttcccagaactacacaacacctagtggagtgataaagtcccccggattccctgaaaaatatcccaacagccttgaatgcacttatattgtctttgcgccaaagatgtcagagattatcctggaatttgaaagctttgacctggagcctgactcaaatcctccaggggggatgttctgtcgctacgaccggctagaaatctgggatggattccctgatgttggccctcacattgggcgttactgtggacagaaaacaccaggtcgaatccgatcctcatcgggcattctctccatggttttttacaccgacagcgcgatagcaaaagaaggtttctcagcaaactacagtgtcttgcagagcagtgtctcagaagatttcaaatgtatggaagctctgggcatggaatcaggagaaattcattctgaccagatcacagcttcttcccagtatagcaccaactggtctgcagagcgctcccgcctgaactaccctgagaatgggtggactcccggagaggattcctaccgagagtggatacaggtagacttgggccttctgcgctttgtcacggctgtcgggacacagggcgccatttcaaaagaaaccaagaagaaatattatgtcaagacttacaagatcgacgttagctccaacggggaagactggatcaccataaaagaaggaaacaaacctgttctctttcagggaaacaccaaccctacagatgttgtggttgcagtattccccaaaccactgataactcgatttgtccgaatcaagcctgcaacttgggaaactggcatatctatgagatttgaagtatatggttgcaagataacagattatcctgaagtggaagcccctacagctggaccgaccactcccaacgggaacttggtggatgaatgtgatgacgaccaggccaactgccacagtggaacaggtgatgacttccagctcacaggtggcaccactgtgctggccacagaaaagcccacggtcatagacagcaccatacaatcagagtttccaacatatggttttaactgtgaatttggctggggctctcacaagaccttctgccactgggaacatgacaatcacgtgcagctcaagtggagtgtgttgaccagcaagacgggacccattcaggatcacacaggagatggcaacttcatctattcccaagctgacgaaaatcagaagggcaaagtggctcgcctggtgagccctgtggtttattcccagaactctgcccactgcatgaccttctggtatcacatgtctgggtcccacgtcggcacactcagggtcaaactgcgctaccagaagccagaggagtacgatcagctggtctggatggccattggacaccaaggtgaccactggaaggaagggcgtgtcttgctccacaagtctctgaaactttatcaggtgattttcgagggcgaaatcggaaaaggaaaccttggtgggattgctgtggatgacattagtattaataaccacatttcacaagaagattgtgcaaaaccagcagacctggataaaaagaacccagaaattaaaattgatgaaacagggagcacgccaggatacgaaggtgaaggagaaggtgacaagaacatctccaggaagccaggcaatgtgttgaagaccttagaccccagatctggatccaaggaaaacttgtatttccagggc

SEQ ID NO: 88 - protein, 694 aa, artificial sequence
  Synthetic construct
FRNDKCGDTIKIESPGYLTSPGYPHSYHPSEKCEWLIQAPDPYQRIMINFNPHFDLEDRDCKYDYVEVFDGENENGHFRGKFCGKIAPPPVVSSGPFLFIKFVSDYETHGAGFSIRYELFKRGPECSQNYTTPSGVIKSPGFPEKYPNSLECTYIVFAPKMSEIILEFESFDLEPDSNPPGGMFCRYDRLEIWDGFPDVGPHIGRYCGQKTPGRIRSSSGILSMVFYTDSAIAKEGFSANYSVLQSSVSEDFKCMEALGMESGEIHSDQITASSQYSTNWSAERSRLNYPENGWTPGEDSYREWIQVDLGLLRFVTAVGTQGAISKETKKKYYVKTYKIDVSSNGEDWITIKEGNKPVLFQGNTNPTDVVVAVFPKPLITRFVRIKPATWETGISMRFEVYGCKITDYPEVEAPTAGPTTPNGNLVDECDDDQANCHSGTGDDFQLTGGTTVLATEKPTVIDSTIQSEFPTYGFNCEFGWGSHKTFCHWEHDNHVQLKWSVLTSKTGPIQDHTGDGNFIYSQADENQKGKVARLVSPVVYSQNSAHCMTFWYHMSGSHVGTLRVKLRYQKPEEYDQLVWMAIGHQGDHWKEGRVLLHKSLKLYQVIFEGEIGKGNLGGIAVDDISINNHISQEDCAKPADLDKKNPEIKIDETGSTPGYEGEGEGDKNISRKPGNVLKTLDPRSGSKENLYFQG

SEQ ID NO: 89 - DNA, 2145 bp, artificial sequence
  Synthetic construct
atggagagggggctgccgctcctctgcgccgtgctcgccctcgtcctcgccccggccggcgcttttcgcaacgataaatgtggcgatactataaaaattgaaagccccgggtaccttacatctcctggttatcctcattcttatcacccaagtgaaaaatgcgaatggctgattcaggctccggacccataccagagaattatgatcaacttcaaccctcacttcgatttggaggacagagactgcaagtatgactacgtggaagtcttcgatggagaaaatgaaaatggacattttaggggaaagttctgtggaaagatagcccctcctcctgttgtgtcttcagggccatttctttttatcaaatttgtctctgactacgaaacacatggtgcaggattttccatacgttatgaacttttcaagagaggtcctgaatgttcccagaactacacaacacctagtggagtgataaagtcccccggattccctgaaaaatatcccaacagccttgaatgcacttatattgtctttgcgccaaagatgtcagagattatcctggaatttgaaagctttgacctggagcctgactcaaatcctccaggggggatgttctgtcgctacgaccggctagaaatctgggatggattccctgatgttggccctcacattgggcgttactgtggacagaaaacaccaggtcgaatccgatcctcatcgggcattctctccatggttttttacaccgacagcgcgatagcaaaagaaggtttctcagcaaactacagtgtcttgcagagcagtgtctcagaagatttcaaatgtatggaagctctgggcatggaatcaggagaaattcattctgaccagatcacagcttcttcccaggctagcaccaactggtctgcagagcgctcccgcctgaactaccctgagaatgggtggactcccggagaggattcctaccgagagtggatacaggtagacttgggccttctgcgctttgtcacggctgtcgggacacagggcgccatttcaaaagaaaccaagaagaaatattatgtcaagacttacaagatcgacgttagctccaacggggaagactggatcaccataaaagaaggaaacaaacctgttctctttcagggaaacaccaaccctacagatgttgtggttgcagtattccccaaaccactgataactcgatttgtccgaatcaagcctgcaacttgggaaactggcatatctatgagatttgaagtatatggttgcaagataacagattatcctgaagtggaagcccctacagctggaccgaccactcccaacgggaacttggtggatgaatgtgatgacgaccaggccaactgccacagtggaacaggtgatgacttccagctcacaggtggcaccactgtgctggccacagaaaagcccacggtcatagacagcaccatacaatcagagtttccaacatatggttttaactgtgaatttggctggggctctcacaagaccttctgccactgggaacatgacaatcacgtgcagctcaagtggagtgtgttgaccagcaagacgggacccattcaggatcacacaggagatggcaacttcatctattcccaagctgacgaaaatcagaagggcaaagtggctcgcctggtgagccctgtggtttattcccagaactctgcccactgcatgaccttctggtatcacatgtctgggtcccacgtcggcacactcagggtcaaactgcgctaccagaagccagaggagtacgatcagctggtctggatggccattggacaccaaggtgaccactggaaggaagggcgtgtcttgctccacaagtctctgaaactttatcaggtgattttcgagggcgaaatcggaaaaggaaaccttggtgggattgctgtggatgacattagtattaataaccacatttcacaagaagattgtgcaaaaccagcagacctggataaaaagaacccagaaattaaaattgatgaaacagggagcacgccaggatacgaaggtgaaggagaaggtgacaagaacatctccaggaagccaggcaatgtgttgaagaccttagaccccagatctggatccaaggaaaacttgtatttccagggc

SEQ ID NO: 90 - protein, 694 aa, artificial sequence
  Synthetic construct
FRNDKCGDTIKIESPGYLTSPGYPHSYHPSEKCEWLIQAPDPYQRIMINFNPHFDLEDRDCKYDYVEVFDGENENGHFRGKFCGKIAPPPVVSSGPFLFIKFVSDYETHGAGFSIRYELFKRGPECSQNYTTPSGVIKSPGFPEKYPNSLECTYIVFAPKMSEIILEFESFDLEPDSNPPGGMFCRYDRLEIWDGFPDVGPHIGRYCGQKTPGRIRSSSGILSMVFYTDSAIAKEGFSANYSVLQSSVSEDFKCMEALGMESGEIHSDQITASSQASTNWSAERSRLNYPENGWTPGEDSYREWIQVDLGLLRFVTAVGTQGAISKETKKKYYVKTYKIDVSSNGEDWITIKEGNKPVLFQGNTNPTDVVVAVFPKPLITRFVRIKPATWETGISMRFEVYGCKITDYPEVEAPTAGPTTPNGNLVDECDDDQANCHSGTGDDFQLTGGTTVLATEKPTVIDSTIQSEFPTYGFNCEFGWGSHKTFCHWEHDNHVQLKWSVLTSKTGPIQDHTGDGNFIYSQADENQKGKVARLVSPVVYSQNSAHCMTFWYHMSGSHVGTLRVKLRYQKPEEYDQLVWMAIGHQGDHWKEGRVLLHKSLKLYQVIFEGEIGKGNLGGIAVDDISINNHISQEDCAKPADLDKKNPEIKIDETGSTPGYEGEGEGDKNISRKPGNVLKTLDPRSGSKENLYFQG

SEQ ID NO: 91 - DNA, 1677 bp, artificial sequence
  Synthetic construct
atggagagggggctgccgctcctctgcgccgtgctcgccctcgtcctcgccccggccggcgcttttcgcaacgataaatgtggcgatactataaaaattgaaagccccgggtaccttacatctcctggttatcctcattcttatcacccaagtgaaaaatgcgaatggctgattcaggctccggacccataccagagaattatgatcaacttcaaccctcacttcgatttggaggacagagactgcaagtatgactacgtggaagtcttcgatggagaaaatgaaaatggacattttaggggaaagttctgtggaaagatagcccctcctcctgttgtgtcttcagggccatttctttttatcaaatttgtctctgactacgaaacacatggtgcaggattttccatacgttatgaacttttcaagagaggtcctgaatgttcccagaactacacaacacctagtggagtgataaagtcccccggattccctgaaaaatatcccaacagccttgaatgcacttatattgtctttgcgccaaagatgtcagagattatcctggaatttgaaagctttgacctggagcctgactcaaatcctccaggggggatgttctgtcgctacgaccggctagaaatctgggatggattccctgatgttggccctcacattgggcgttactgtggacagaaaacaccaggtcgaatccgatcctcatcgggcattctctccatggttttttacaccgacagcgcgatagcaaaagaaggtttctcagcaaactacagtgtcttgcagagcagtgtctcagaagatttcaaagaagtggaagcccctacagctggaccgaccactcccaacgggaacttggtggatgaatgtgatgacgaccaggccaactgccacagtggaacaggtgatgacttccagctcacaggtggcaccactgtgctggccacagaaaagcccacggtcatagacagcaccatacaatcagagtttccaacatatggttttaactgtgaatttggctggggctctcacaagaccttctgccactgggaacatgacaatcacgtgcagctcaagtggagtgtgttgaccagcaagacgggacccattcaggatcacacaggagatggcaacttcatctattcccaagctgacgaaaatcagaagggcaaagtggctcgcctggtgagccctgtggtttattcccagaactctgcccactgcatgaccttctggtatcacatgtctgggtcccacgtcggcacactcagggtcaaactgcgctaccagaagccagaggagtacgatcagctggtctggatggccattggacaccaaggtgaccactggaaggaagggcgtgtcttgctccacaagtctctgaaactttatcaggtgattttcgagggcgaaatcggaaaaggaaaccttggtgggattgctgtggatgacattagtattaataaccacatttcacaagaagattgtgcaaaaccagcagacctggataaaaagaacccagaaattaaaattgatgaaacagggagcacgccaggatacgaaggtgaaggagaaggtgacaagaacatctccaggaagccaggcaatgtgttgaagaccttagaccccagatctggatccaaggaaaacttgtatttccagggc

SEQ ID NO: 92 - protein, 538 aa, artificial sequence
  Synthetic construct
FRNDKCGDTIKIESPGYLTSPGYPHSYHPSEKCEWLIQAPDPYQRIMINFNPHFDLEDRDCKYDYVEVFDGENENGHFRGKFCGKIAPPPVVSSGPFLFIKFVSDYETHGAGFSIRYELFKRGPECSQNYTTPSGVIKSPGFPEKYPNSLECTYIVFAPKMSEIILEFESFDLEPDSNPPGGMFCRYDRLEIWDGFPDVGPHIGRYCGQKTPGRIRSSSGILSMVFYTDSAIAKEGFSANYSVLQSSVSEDFKEVEAPTAGPTTPNGNLVDECDDDQANCHSGTGDDFQLTGGTTVLATEKPTVIDSTIQSEFPTYGFNCEFGWGSHKTFCHWEHDNHVQLKWSVLTSKTGPIQDHTGDGNFIYSQADENQKGKVARLVSPVVYSQNSAHCMTFWYHMSGSHVGTLRVKLRYQKPEEYDQLVWMAIGHQGDHWKEGRVLLHKSLKLYQVIFEGEIGKGNLGGIAVDDISINNHISQEDCAKPADLDKKNPEIKIDETGSTPGYEGEGEGDKNISRKPGNVLKTLDPRSGSKENLYFQG

SEQ ID NO: 93 - DNA, 2115 bp, artificial sequence
  Synthetic construct
atggagagggggctgccgctcctctgcgccgtgctcgccctcgtcctcgccccggccggcgcttttcgcaacgataaatgtggcgatactataaaaattgaaagccccgggtaccttacatctcctggttatcctcattcttatcacccaagtgaaaaatgcgaatggctgattcaggctccggacccataccagagaattatgatcaacttcaaccctcacttcgatttggaggacagagactgcaagtatgactacgtggaagtcttcgatggagaaaatgaaaatggacattttaggggaaagttctgtggaaagatagcccctcctcctgttgtgtcttcagggccatttctttttatcaaatttgtctctgactacgaaacacatggtgcaggattttccatacgttatgaacttttcaagagaggtcctgaatgttcccagaactacacaacacctagtggagtgataaagtcccccggattccctgaaaaatatcccaacagccttgaatgcacttatattgtctttgcgccaaagatgtcagagattatcctggaatttgaaagctttgacctggagcctgactcaaatcctccaggggggatgttctgtcgctacgaccggctagaaatctgggatggattccctgatgttggccctcacattgggcgttactgtggacagaaaacaccaggtcgaatccgatcctcatcgggcattctctccatggttttttacaccgacagcgcgatagcaaaagaaggtttctcagcaaactacagtgtcttgcagagcagtgtctcagaagatttcaaatgtatggaagctctgggcatggaatcaggagaaattcattctgaccagatcacagcttcttcccagtatagcaccaactggtctgcagagcgctcccgcctgaactaccctgagaatgggtggactcccggagaggattcctaccgagagtggatacaggtagacttgggccttctgcgctttgtcacggctgtcgggacacagggcgccatttcaaaagaaaccaagaagaaatattatgtcaagacttacaagatcgacgttagctccaacggggaagactggatcaccataaaagaaggaaacaaacctgttctctttcagggaaacaccaaccctacagatgttgtggttgcagtattccccaaaccactgataactcgatttgtccgaatcaagcctgcaacttgggaaactggcatatctatgagatttgaagtatatggttgcaagataacagattatcctgaagtggaagcccctacagctggaccgaccactcccaacgggaacttggtggatgaatgtgatgacgaccaggccaactgccacagtggaacaggtgatgacttccagctcacaggtggcaccactgtgctggccacagaaaagcccacggtcatagacagcaccatacaatcagagtttccaacatatggttttaactgtgaatttggctggggctctcacaagaccttctgccactgggaacatgacaatcacgtgcagctcaagtggagtgtgttgaccagcaagacgggacccattcaggatcacacaggagatggcaacttcatctattcccaagctgacgaaaatcagaagggcaaagtggctcgcctggtgagccctgtggtttattcccagaactctgcccactgcatgaccttctggtatcacatgtctgggtcccacgtcggcacactcagggtcaaactgcgctaccagaagccagaggagtacgatcagctggtctggatggccattggacaccaaggtgaccactggaaggaagggcgtgtcttgctccacaagtctctgaaactttatcaggtgattttcgagggcgaaatcggaaaaggaaaccttggtgggattgctgtggatgacattagtattaataaccacatttcacaagaagattgtgcaaaaccagcagacctggataaaaagaacccagaaattaaaattgatgaaacagggagcacgccaggatacgaaggtgaaggagaaggtgacaagaacatctccaggaagccaggcaatgtgttgaagaccttagaccccagatct

SEQ ID NO: 94 - protein, 682 aa, artificial sequence
  Synthetic construct
FRNDKCGDTIKIESPGYLTSPGYPHSYHPSEKCEWLIQAPDPYQRIMINFNPHFDLEDRDCKYDYVEVFDGENENGHFRGKFCGKIAPPPVVSSGPFLFIKFVSDYETHGAGFSIRYELFKRGPECSQNYTTPSGVIKSPGFPEKYPNSLECTYIVFAPKMSEIILEFESFDLEPDSNPPGGMFCRYDRLEIWDGFPDVGPHIGRYCGQKTPGRIRSSSGILSMVFYTDSAIAKEGFSANYSVLQSSVSEDFKCMEALGMESGEIHSDQITASSQYSTNWSAERSRLNYPENGWTPGEDSYREWIQVDLGLLRFVTAVGTQGAISKETKKKYYVKTYKIDVSSNGEDWITIKEGNKPVLFQGNTNPTDVVVAVFPKPLITRFVRIKPATWETGISMRFEVYGCKITDYPEVEAPTAGPTTPNGNLVDECDDDQANCHSGTGDDFQLTGGTTVLATEKPTVIDSTIQSEFPTYGFNCEFGWGSHKTFCHWEHDNHVQLKWSVLTSKTGPIQDHTGDGNFIYSQADENQKGKVARLVSPVVYSQNSAHCMTFWYHMSGSHVGTLRVKLRYQKPEEYDQLVWMAIGHQGDHWKEGRVLLHKSLKLYQVIFEGEIGKGNLGGIAVDDISINNHISQEDCAKPADLDKKNPEIKIDETGSTPGYEGEGEGDKNISRKPGNVLKTLDP

SEQ ID NO: 95 - protein, 923 aa, artificial sequence
  Synthetic construct
MERGLPLLCATLALALALAGAFRSDKCGGTIKIENPGYLTSPGYPHSYHPSEKCEWLIQAPEPYQRIMINFNPHFDLEDRDCKYDYVEVIDGENEGGRLWGKFCGKIAPSPVVSSGPFLFIKFVSDYETHGAGFSIRYEIFKRGPECSQNYTAPTGVIKSPGFPEKYPNSLECTYIIFAPKMSEIILEFESFDLEQDSNPPGGVFCRYDRLEIWDGFPEVGPHIGRYCGQKTPGRIRSSSGILSMVFYTDSAIAKEGFSANYSVLQSSISEDFKCMEALGMESGEIHSDQITASSQYGTNWSVERSRLNYPENGWTPGEDSYREWIQVDLGLLRFVTAVGTQGAISKETKKKYYVKTYRVDISSNGEDWITLKEGNKAIIFQGNTNPTDVVFGVFPKPLITRFVRIKPASWETGISMRFEVYGCKITDYPCSGMLGMVSGLISDSQITASNQGDRNWMPENIRLVTSRTGWALPPSPHPYINEWLQVDLGDEKIVRGVIIQGGKHRENKVFMRKFKIAYSNNGSDWKMIMDDSKRKAKSFEGNNNYDTPELRAFTPLSTRFIRIYPERATHSGLGLRMELLGCEVEVPTAGPTTPNGNPVDECDDDQANCHSGTGDDFQLTGGTTVLATEKPTIIDSTIQSEFPTYGFNCEFGWGSHKTFCHWEHDSHAQLRWRVLTSKTGPIQDHTGDGNFIYSQADENQKGKVARLVSPVVYSQSSAHCMTFWYHMSGSHVGTLRVKLHYQKPEEYDQLVWMVVGHQGDHWKEGRVLLHKSLKLYQVIFEGEIGKGNLGGIAVDDISINNHIPQEDCAKPTDLDKKNTEIKIDETGSTPGYEEEGKGDKNISRKPGNVLKTLDPILITIIAMSALGVLLGAVCGVVLYCACWHNGMSERNLSALENYNFELVDGVKLKKDKLNPQSNYSEA

SEQ ID NO: 96 - protein, 923 aa, artificial sequence [sequence omitted]

SEQ ID NO: 97 - protein, 7 aa, artificial sequence
  Synthetic construct
  VARIANT (2)..(2): X can be any amino acid
  VARIANT (3)..(3): X can be any amino acid
  VARIANT (5)..(5): X can be any amino acid
EXXYXQG

SEQ ID NO: 98 - protein, 7 aa, artificial sequence
  Synthetic construct
  VARIANT (2)..(2): X is any amino acid
  VARIANT (3)..(3): X is any amino acid
  VARIANT (5)..(5): X is any amino acid
EXXYXQS

SEQ ID NO: 99 - DNA, 20 bp, Artificial Sequence
  NRP1 forward primer
acccacatttcgatttggag

SEQ ID NO: 100 - DNA, 20 bp, Artificial Sequence
  NRP1 reverse primer
ttcatagcggatggaaaacc

SEQ ID NO: 101 - DNA, 20 bp, Artificial Sequence
  SEMA3A forward primer
gctcctgctccgtagcctgc

SEQ ID NO: 102 - DNA, 20 bp, Artificial Sequence
  SEMA3A Reverse primer
tcggcgttgctttcggtccc

SEQ ID NO: 103 - DNA, 14 bp, Artificial Sequence
  SEMA3e forward primer
tctgcaaccatcca

SEQ ID NO: 104 - DNA, 22 bp, Artificial Sequence
  SEMA3e reverse primer
accacaagagggaagcacagac

SEQ ID NO: 105 - DNA, 20 bp, Artificial Sequence
  TGFb forward primer
ggactctccacctgcaagac

SEQ ID NO: 106 - DNA, 20 bp, Artificial Sequence
  TGFb reverse primer
catagatggcgttgttgcgg

SEQ ID NO: 107 - DNA, 20 bp, Artificial Sequence
  VEGFa forward primer
gccctgagtcaagaggacag

SEQ ID NO: 108 - DNA, 20 bp, Artificial Sequence
  VEGFa reverse primer
ctcctaggcccctcagaagt

SEQ ID NO: 109 - DNA, 20 bp, Artificial Sequence
  VEGFb forward primer
tctgagcatggaactcatgg

SEQ ID NO: 110 - DNA, 20 bp, Artificial Sequence
  VEGFb reverse primer
tctgcattcacattggctgt